European Patent Application EP 4 807 000 A1, published September 16, 2026. Title: 一种通用的制备环状RNA的方法及其用途. Applicant: 上海元码智药生物技术有限公司. The sequence listing filed with the application follows.

SEQUENCE LISTING (90 sequences)

SEQ ID NO: 1 - RNA, 741 nt, synthetic construct
  source 1..741: mol_type = other RNA
ttaaaacagcctgtgggttgatcccacccacaggcccattgggcgctagcactctggtatcacggtacctttgtgcgcctgttttataccccctcccccaactgtaacttagaagtaacacacaccgatcaacagtcagcgtggcacaccagccacgttttgatcaagcacttctgttaccccggactgagtatcaatagactgctcacgcggttgaaggagaaagcgttcgttatccggccaactacttcgaaaaacctagtaacaccgtggaagttgcagagtgtttcgctcagcactaccccagtgtagatcaggtcgatgagtcaccgcattccccacgggcgaccgtggcggtggctgcgttggcggcctgcccatggggaaacccatgggacgctctaatacagacatggtgcgaagagtctattgagctagttggtagtcctccggcccctgaatgcggctaatcctaactgcggagcacacaccctcaagccagagggcagtgtgtcgtaacgggcaactctgcagcggaaccgactactttgggtgtccgtgtttcattttattcctatactggctgcttatggtgacaattgagagatcgttaccatatagctattggattggccatccggtgactaatagagctattatatatccctttgttgggtttataccacttagcttgaaagaggttaaaacattacaattcattgttaagttgaatacagcaaa

SEQ ID NO: 2 - RNA, 94 nt, synthetic construct
  source 1..94: mol_type = other RNA
ttaaaacagcctgtgggttgatcccacccacaggcccattgggcgctagcactctggtatcacggtacctttgtgcgcctgttttataccccct

SEQ ID NO: 3 - RNA, 558 nt, synthetic construct
  source 1..558: mol_type = other RNA
atgggagtcaaagttctgtttgccctgatctgcatcgctgtggccgaggccaagcccaccgagaacaacgaagacttcaacatcgtggccgtggccagcaacttcgcgaccacggatctcgatgctgaccgcgggaagttgcccggcaagaagctgccgctggaggtgctcaaagagatggaagccaatgcccggaaagctggctgcaccaggggctgtctgatctgcctgtcccacatcaagtgcacgcccaagatgaagaagttcatcccaggacgctgccacacctacgaaggcgacaaagagtccgcacagggcggcataggcgaggcgatcgtcgacattcctgagattcctgggttcaaggacttggagcccatggagcagttcatcgcacaggtcgatctgtgtgtggactgcacaactggctgcctcaaagggcttgccaacgtgcagtgttctgacctgctcaagaagtggctgccgcaacgctgtgcgacctttgccagcaagatccagggccaggtggacaagatcaagggggccggtggtgactaa

SEQ ID NO: 4 - RNA, 1299 nt, synthetic construct
  source 1..1299: mol_type = other RNA
ttaaaacagcctgtgggttgatcccacccacaggcccattgggcgctagcactctggtatcacggtacctttgtgcgcctgttttataccccctcccccaactgtaacttagaagtaacacacaccgatcaacagtcagcgtggcacaccagccacgttttgatcaagcacttctgttaccccggactgagtatcaatagactgctcacgcggttgaaggagaaagcgttcgttatccggccaactacttcgaaaaacctagtaacaccgtggaagttgcagagtgtttcgctcagcactaccccagtgtagatcaggtcgatgagtcaccgcattccccacgggcgaccgtggcggtggctgcgttggcggcctgcccatggggaaacccatgggacgctctaatacagacatggtgcgaagagtctattgagctagttggtagtcctccggcccctgaatgcggctaatcctaactgcggagcacacaccctcaagccagagggcagtgtgtcgtaacgggcaactctgcagcggaaccgactactttgggtgtccgtgtttcattttattcctatactggctgcttatggtgacaattgagagatcgttaccatatagctattggattggccatccggtgactaatagagctattatatatccctttgttgggtttataccacttagcttgaaagaggttaaaacattacaattcattgttaagttgaatacagcaaaatgggagtcaaagttctgtttgccctgatctgcatcgctgtggccgaggccaagcccaccgagaacaacgaagacttcaacatcgtggccgtggccagcaacttcgcgaccacggatctcgatgctgaccgcgggaagttgcccggcaagaagctgccgctggaggtgctcaaagagatggaagccaatgcccggaaagctggctgcaccaggggctgtctgatctgcctgtcccacatcaagtgcacgcccaagatgaagaagttcatcccaggacgctgccacacctacgaaggcgacaaagagtccgcacagggcggcataggcgaggcgatcgtcgacattcctgagattcctgggttcaaggacttggagcccatggagcagttcatcgcacaggtcgatctgtgtgtggactgcacaactggctgcctcaaagggcttgccaacgtgcagtgttctgacctgctcaagaagtggctgccgcaacgctgtgcgacctttgccagcaagatccagggccaggtggacaagatcaagggggccggtggtgactaa

SEQ ID NO: 5 - RNA, 1299 nt, synthetic construct
  source 1..1299: mol_type = other RNA
cccacccacaggcccattgggcgctagcactctggtatcacggtacctttgtgcgcctgttttataccccctcccccaactgtaacttagaagtaacacacaccgatcaacagtcagcgtggcacaccagccacgttttgatcaagcacttctgttaccccggactgagtatcaatagactgctcacgcggttgaaggagaaagcgttcgttatccggccaactacttcgaaaaacctagtaacaccgtggaagttgcagagtgtttcgctcagcactaccccagtgtagatcaggtcgatgagtcaccgcattccccacgggcgaccgtggcggtggctgcgttggcggcctgcccatggggaaacccatgggacgctctaatacagacatggtgcgaagagtctattgagctagttggtagtcctccggcccctgaatgcggctaatcctaactgcggagcacacaccctcaagccagagggcagtgtgtcgtaacgggcaactctgcagcggaaccgactactttgggtgtccgtgtttcattttattcctatactggctgcttatggtgacaattgagagatcgttaccatatagctattggattggccatccggtgactaatagagctattatatatccctttgttgggtttataccacttagcttgaaagaggttaaaacattacaattcattgttaagttgaatacagcaaaatgggagtcaaagttctgtttgccctgatctgcatcgctgtggccgaggccaagcccaccgagaacaacgaagacttcaacatcgtggccgtggccagcaacttcgcgaccacggatctcgatgctgaccgcgggaagttgcccggcaagaagctgccgctggaggtgctcaaagagatggaagccaatgcccggaaagctggctgcaccaggggctgtctgatctgcctgtcccacatcaagtgcacgcccaagatgaagaagttcatcccaggacgctgccacacctacgaaggcgacaaagagtccgcacagggcggcataggcgaggcgatcgtcgacattcctgagattcctgggttcaaggacttggagcccatggagcagttcatcgcacaggtcgatctgtgtgtggactgcacaactggctgcctcaaagggcttgccaacgtgcagtgttctgacctgctcaagaagtggctgccgcaacgctgtgcgacctttgccagcaagatccagggccaggtggacaagatcaagggggccggtggtgactaattaaaacagcctgtgggttgat

SEQ ID NO: 6 - RNA, 165 nt, synthetic construct
  source 1..165: mol_type = other RNA
gggtcacccgtcgcgcggtttggtatactaggccaacaatagatgacttacaactaatcggaaggtgcagagactcgacgggagctaccctaacgtcaagacgagggtaaagagagagtccaattctcaaagccaataggcagtagcgaaagctgcaagagaatg

SEQ ID NO: 7 - RNA, 151 nt, synthetic construct
  source 1..151: mol_type = other RNA
aaataattgtcccttaaagaagaaattctttaagtggatgctctcaaactcagggaaacctaaatctagttatagacaaggcaatcctgagccaagccgaagtagtaattagtaaggcctagtataccaaaccgcgatatctcttttctag

SEQ ID NO: 8 - RNA, 1615 nt, synthetic construct
  source 1..1615: mol_type = other RNA
gggtcacccgtcgcgcggtttggtatactaggccaacaatagatgacttacaactaatcggaaggtgcagagactcgacgggagctaccctaacgtcaagacgagggtaaagagagagtccaattctcaaagccaataggcagtagcgaaagctgcaagagaatgcccacccacaggcccattgggcgctagcactctggtatcacggtacctttgtgcgcctgttttataccccctcccccaactgtaacttagaagtaacacacaccgatcaacagtcagcgtggcacaccagccacgttttgatcaagcacttctgttaccccggactgagtatcaatagactgctcacgcggttgaaggagaaagcgttcgttatccggccaactacttcgaaaaacctagtaacaccgtggaagttgcagagtgtttcgctcagcactaccccagtgtagatcaggtcgatgagtcaccgcattccccacgggcgaccgtggcggtggctgcgttggcggcctgcccatggggaaacccatgggacgctctaatacagacatggtgcgaagagtctattgagctagttggtagtcctccggcccctgaatgcggctaatcctaactgcggagcacacaccctcaagccagagggcagtgtgtcgtaacgggcaactctgcagcggaaccgactactttgggtgtccgtgtttcattttattcctatactggctgcttatggtgacaattgagagatcgttaccatatagctattggattggccatccggtgactaatagagctattatatatccctttgttgggtttataccacttagcttgaaagaggttaaaacattacaattcattgttaagttgaatacagcaaaatgggagtcaaagttctgtttgccctgatctgcatcgctgtggccgaggccaagcccaccgagaacaacgaagacttcaacatcgtggccgtggccagcaacttcgcgaccacggatctcgatgctgaccgcgggaagttgcccggcaagaagctgccgctggaggtgctcaaagagatggaagccaatgcccggaaagctggctgcaccaggggctgtctgatctgcctgtcccacatcaagtgcacgcccaagatgaagaagttcatcccaggacgctgccacacctacgaaggcgacaaagagtccgcacagggcggcataggcgaggcgatcgtcgacattcctgagattcctgggttcaaggacttggagcccatggagcagttcatcgcacaggtcgatctgtgtgtggactgcacaactggctgcctcaaagggcttgccaacgtgcagtgttctgacctgctcaagaagtggctgccgcaacgctgtgcgacctttgccagcaagatccagggccaggtggacaagatcaagggggccggtggtgactaattaaaacagcctgtgggttgataaataattgtcccttaaagaagaaattctttaagtggatgctctcaaactcagggaaacctaaatctagttatagacaaggcaatcctgagccaagccgaagtagtaattagtaaggcctagtataccaaaccgcgatatctcttttctag

SEQ ID NO: 9 - RNA, 151 nt, synthetic construct
  source 1..151: mol_type = other RNA
aaataattgagccttaaagaagaaattctttaagtggatgctctcaaactcagggaaacctaaatctagttatagacaaggcaatcctgagccaagccgaagtagtaattagtaaggcctagtataccaaaccgcgatatctcttttctag

SEQ ID NO: 10 - RNA, 1615 nt, synthetic construct
  source 1..1615: mol_type = other RNA
gggtcacccgtcgcgcggtttggtatactaggccaacaatagatgacttacaactaatcggaaggtgcagagactcgacgggagctaccctaacgtcaagacgagggtaaagagagagtccaattctcaaagccaataggcagtagcgaaagctgcaagagaatgcccacccacaggcccattgggcgctagcactctggtatcacggtacctttgtgcgcctgttttataccccctcccccaactgtaacttagaagtaacacacaccgatcaacagtcagcgtggcacaccagccacgttttgatcaagcacttctgttaccccggactgagtatcaatagactgctcacgcggttgaaggagaaagcgttcgttatccggccaactacttcgaaaaacctagtaacaccgtggaagttgcagagtgtttcgctcagcactaccccagtgtagatcaggtcgatgagtcaccgcattccccacgggcgaccgtggcggtggctgcgttggcggcctgcccatggggaaacccatgggacgctctaatacagacatggtgcgaagagtctattgagctagttggtagtcctccggcccctgaatgcggctaatcctaactgcggagcacacaccctcaagccagagggcagtgtgtcgtaacgggcaactctgcagcggaaccgactactttgggtgtccgtgtttcattttattcctatactggctgcttatggtgacaattgagagatcgttaccatatagctattggattggccatccggtgactaatagagctattatatatccctttgttgggtttataccacttagcttgaaagaggttaaaacattacaattcattgttaagttgaatacagcaaaatgggagtcaaagttctgtttgccctgatctgcatcgctgtggccgaggccaagcccaccgagaacaacgaagacttcaacatcgtggccgtggccagcaacttcgcgaccacggatctcgatgctgaccgcgggaagttgcccggcaagaagctgccgctggaggtgctcaaagagatggaagccaatgcccggaaagctggctgcaccaggggctgtctgatctgcctgtcccacatcaagtgcacgcccaagatgaagaagttcatcccaggacgctgccacacctacgaaggcgacaaagagtccgcacagggcggcataggcgaggcgatcgtcgacattcctgagattcctgggttcaaggacttggagcccatggagcagttcatcgcacaggtcgatctgtgtgtggactgcacaactggctgcctcaaagggcttgccaacgtgcagtgttctgacctgctcaagaagtggctgccgcaacgctgtgcgacctttgccagcaagatccagggccaggtggacaagatcaagggggccggtggtgactaattaaaacagcctgtgggttgataaataattgagccttaaagaagaaattctttaagtggatgctctcaaactcagggaaacctaaatctagttatagacaaggcaatcctgagccaagccgaagtagtaattagtaaggcctagtataccaaaccgcgatatctcttttctag

SEQ ID NO: 11 - RNA, 1615 nt, synthetic construct
  source 1..1615: mol_type = other RNA
gggtcacccgtcgcgcggtttggtatactaggccaacaatagatgacttacaactaatcggaaggtgcagagactcgacgggagctaccctaacgtcaagacgagggtaaagagagagtccaattctcaaagccaataggcagtagcgaaagctgcaagagaatggatcccacccacaggcccattgggcgctagcactctggtatcacggtacctttgtgcgcctgttttataccccctcccccaactgtaacttagaagtaacacacaccgatcaacagtcagcgtggcacaccagccacgttttgatcaagcacttctgttaccccggactgagtatcaatagactgctcacgcggttgaaggagaaagcgttcgttatccggccaactacttcgaaaaacctagtaacaccgtggaagttgcagagtgtttcgctcagcactaccccagtgtagatcaggtcgatgagtcaccgcattccccacgggcgaccgtggcggtggctgcgttggcggcctgcccatggggaaacccatgggacgctctaatacagacatggtgcgaagagtctattgagctagttggtagtcctccggcccctgaatgcggctaatcctaactgcggagcacacaccctcaagccagagggcagtgtgtcgtaacgggcaactctgcagcggaaccgactactttgggtgtccgtgtttcattttattcctatactggctgcttatggtgacaattgagagatcgttaccatatagctattggattggccatccggtgactaatagagctattatatatccctttgttgggtttataccacttagcttgaaagaggttaaaacattacaattcattgttaagttgaatacagcaaaatgggagtcaaagttctgtttgccctgatctgcatcgctgtggccgaggccaagcccaccgagaacaacgaagacttcaacatcgtggccgtggccagcaacttcgcgaccacggatctcgatgctgaccgcgggaagttgcccggcaagaagctgccgctggaggtgctcaaagagatggaagccaatgcccggaaagctggctgcaccaggggctgtctgatctgcctgtcccacatcaagtgcacgcccaagatgaagaagttcatcccaggacgctgccacacctacgaaggcgacaaagagtccgcacagggcggcataggcgaggcgatcgtcgacattcctgagattcctgggttcaaggacttggagcccatggagcagttcatcgcacaggtcgatctgtgtgtggactgcacaactggctgcctcaaagggcttgccaacgtgcagtgttctgacctgctcaagaagtggctgccgcaacgctgtgcgacctttgccagcaagatccagggccaggtggacaagatcaagggggccggtggtgactaattaaaacagcctgtgggttaaataattgacccttaaagaagaaattctttaagtggatgctctcaaactcagggaaacctaaatctagttatagacaaggcaatcctgagccaagccgaagtagtaattagtaaggcctagtataccaaaccgcgatatctcttttctag

SEQ ID NO: 12 - RNA, 1615 nt, synthetic construct
  source 1..1615: mol_type = other RNA
gggtcacccgtcgcgcggtttggtatactaggccaacaatagatgacttacaactaatcggaaggtgcagagactcgacgggagctaccctaacgtcaagacgagggtaaagagagagtccaattctcaaagccaataggcagtagcgaaagctgcaagagaatggggcgctagcactctggtatcacggtacctttgtgcgcctgttttataccccctcccccaactgtaacttagaagtaacacacaccgatcaacagtcagcgtggcacaccagccacgttttgatcaagcacttctgttaccccggactgagtatcaatagactgctcacgcggttgaaggagaaagcgttcgttatccggccaactacttcgaaaaacctagtaacaccgtggaagttgcagagtgtttcgctcagcactaccccagtgtagatcaggtcgatgagtcaccgcattccccacgggcgaccgtggcggtggctgcgttggcggcctgcccatggggaaacccatgggacgctctaatacagacatggtgcgaagagtctattgagctagttggtagtcctccggcccctgaatgcggctaatcctaactgcggagcacacaccctcaagccagagggcagtgtgtcgtaacgggcaactctgcagcggaaccgactactttgggtgtccgtgtttcattttattcctatactggctgcttatggtgacaattgagagatcgttaccatatagctattggattggccatccggtgactaatagagctattatatatccctttgttgggtttataccacttagcttgaaagaggttaaaacattacaattcattgttaagttgaatacagcaaaatgggagtcaaagttctgtttgccctgatctgcatcgctgtggccgaggccaagcccaccgagaacaacgaagacttcaacatcgtggccgtggccagcaacttcgcgaccacggatctcgatgctgaccgcgggaagttgcccggcaagaagctgccgctggaggtgctcaaagagatggaagccaatgcccggaaagctggctgcaccaggggctgtctgatctgcctgtcccacatcaagtgcacgcccaagatgaagaagttcatcccaggacgctgccacacctacgaaggcgacaaagagtccgcacagggcggcataggcgaggcgatcgtcgacattcctgagattcctgggttcaaggacttggagcccatggagcagttcatcgcacaggtcgatctgtgtgtggactgcacaactggctgcctcaaagggcttgccaacgtgcagtgttctgacctgctcaagaagtggctgccgcaacgctgtgcgacctttgccagcaagatccagggccaggtggacaagatcaagggggccggtggtgactaattaaaacagcctgtgggttgatcccacccacaggcccattaaataattgatccttaaagaagaaattctttaagtggatgctctcaaactcagggaaacctaaatctagttatagacaaggcaatcctgagccaagccgaagtagtaattagtaaggcctagtataccaaaccgcgatatctcttttctag

SEQ ID NO: 13 - DNA, 20 bp, synthetic construct
  source 1..20: mol_type = other DNA
tgtgcgatgaactgctccat

SEQ ID NO: 14 - DNA, 22 bp, synthetic construct
  source 1..22: mol_type = other DNA
aagaagttcatcccaggacgct

SEQ ID NO: 15 - DNA, 20 bp, synthetic construct
  source 1..20: mol_type = other DNA
ggccacgatgttgaagtctt

SEQ ID NO: 16 - RNA, 1615 nt, synthetic construct
  source 1..1615: mol_type = other RNA
gggtcacccgtcgcgcggtttggtatactaggccaacaatagatgacttacaactaatcggaaggtgcagagactcgacgggagctaccctaacgtcaagacgagggtaaagagagagtccaattctcaaagccaataggcagtagcgaaagctgcaagagaatgcccacccacaggcccattgggcgctagcactctggtatcacggtacctttgtgcgcctgttttataccccctcccccaactgtaacttagaagtaacacacaccgatcaacagtcagcgtggcacaccagccacgttttgatcaagcacttctgttaccccggactgagtatcaatagactgctcacgcggttgaaggagaaagcgttcgttatccggccaactacttcgaaaaacctagtaacaccgtggaagttgcagagtgtttcgctcagcactaccccagtgtagatcaggtcgatgagtcaccgcattccccacgggcgaccgtggcggtggctgcgttggcggcctgcccatggggaaacccatgggacgctctaatacagacatggtgcgaagagtctattgagctagttggtagtcctccggcccctgaatgcggctaatcctaactgcggagcacacaccctcaagccagagggcagtgtgtcgtaacgggcaactctgcagcggaaccgactactttgggtgtccgtgtttcattttattcctatactggctgcttatggtgacaattgagagatcgttaccatatagctattggattggccatccggtgactaatagagctattatatatccctttgttgggtttataccacttagcttgaaagaggttaaaacattacaattcattgttaagttgaatacagcaaaatgggagtcaaagttctgtttgccctgatctgcatcgctgtggccgaggccaagcccaccgagaacaacgaagacttcaacatcgtggccgtggccagcaacttcgcgaccacggatctcgatgctgaccgcgggaagttgcccggcaagaagctgccgctggaggtgctcaaagagatggaagccaatgcccggaaagctggctgcaccaggggctgtctgatctgcctgtcccacatcaagtgcacgcccaagatgaagaagttcatcccaggacgctgccacacctacgaaggcgacaaagagtccgcacagggcggcataggcgaggcgatcgtcgacattcctgagattcctgggttcaaggacttggagcccatggagcagttcatcgcacaggtcgatctgtgtgtggactgcacaactggctgcctcaaagggcttgccaacgtgcagtgttctgacctgctcaagaagtggctgccgcaacgctgtgcgacctttgccagcaagatccagggccaggtggacaagatcaagggggccggtggtgactaattaaaacagcctgtgggttgataaataattgtcaactaaagaagaaattctttaagtggatgctctcaaactcagggaaacctaaatctagttatagacaaggcaatcctgagccaagccgaagtagtaattagtaaggcctagtataccaaaccgcgatatctcttttctag

SEQ ID NO: 17 - RNA, 1615 nt, synthetic construct
  source 1..1615: mol_type = other RNA
gggtcacccgtcgcgcggtttggtatactaggccaacaatagatgacttacaactaatcggaaggtgcagagactcgacgggagctaccctaacgtcaagacgagggtaaagagagagtccaattctcaaagccaataggcagtagcgaaagctgcaagagaatgcccacccacaggcccattgggcgctagcactctggtatcacggtacctttgtgcgcctgttttataccccctcccccaactgtaacttagaagtaacacacaccgatcaacagtcagcgtggcacaccagccacgttttgatcaagcacttctgttaccccggactgagtatcaatagactgctcacgcggttgaaggagaaagcgttcgttatccggccaactacttcgaaaaacctagtaacaccgtggaagttgcagagtgtttcgctcagcactaccccagtgtagatcaggtcgatgagtcaccgcattccccacgggcgaccgtggcggtggctgcgttggcggcctgcccatggggaaacccatgggacgctctaatacagacatggtgcgaagagtctattgagctagttggtagtcctccggcccctgaatgcggctaatcctaactgcggagcacacaccctcaagccagagggcagtgtgtcgtaacgggcaactctgcagcggaaccgactactttgggtgtccgtgtttcattttattcctatactggctgcttatggtgacaattgagagatcgttaccatatagctattggattggccatccggtgactaatagagctattatatatccctttgttgggtttataccacttagcttgaaagaggttaaaacattacaattcattgttaagttgaatacagcaaaatgggagtcaaagttctgtttgccctgatctgcatcgctgtggccgaggccaagcccaccgagaacaacgaagacttcaacatcgtggccgtggccagcaacttcgcgaccacggatctcgatgctgaccgcgggaagttgcccggcaagaagctgccgctggaggtgctcaaagagatggaagccaatgcccggaaagctggctgcaccaggggctgtctgatctgcctgtcccacatcaagtgcacgcccaagatgaagaagttcatcccaggacgctgccacacctacgaaggcgacaaagagtccgcacagggcggcataggcgaggcgatcgtcgacattcctgagattcctgggttcaaggacttggagcccatggagcagttcatcgcacaggtcgatctgtgtgtggactgcacaactggctgcctcaaagggcttgccaacgtgcagtgttctgacctgctcaagaagtggctgccgcaacgctgtgcgacctttgccagcaagatccagggccaggtggacaagatcaagggggccggtggtgactaattaaaacagcctgtgggttgataaataattgtcaacccaagaagaaattctttaagtggatgctctcaaactcagggaaacctaaatctagttatagacaaggcaatcctgagccaagccgaagtagtaattagtaaggcctagtataccaaaccgcgatatctcttttctag

SEQ ID NO: 18 - RNA, 1615 nt, synthetic construct
  source 1..1615: mol_type = other RNA
gggtcacccgtcgcgcggtttggtatactaggccaacaatagatgacttacaactaatcggaaggtgcagagactcgacgggagctaccctaacgtcaagacgagggtaaagagagagtccaattctcaaagccaataggcagtagcgaaagctgcaagagaatgcccacccacaggcccattgggcgctagcactctggtatcacggtacctttgtgcgcctgttttataccccctcccccaactgtaacttagaagtaacacacaccgatcaacagtcagcgtggcacaccagccacgttttgatcaagcacttctgttaccccggactgagtatcaatagactgctcacgcggttgaaggagaaagcgttcgttatccggccaactacttcgaaaaacctagtaacaccgtggaagttgcagagtgtttcgctcagcactaccccagtgtagatcaggtcgatgagtcaccgcattccccacgggcgaccgtggcggtggctgcgttggcggcctgcccatggggaaacccatgggacgctctaatacagacatggtgcgaagagtctattgagctagttggtagtcctccggcccctgaatgcggctaatcctaactgcggagcacacaccctcaagccagagggcagtgtgtcgtaacgggcaactctgcagcggaaccgactactttgggtgtccgtgtttcattttattcctatactggctgcttatggtgacaattgagagatcgttaccatatagctattggattggccatccggtgactaatagagctattatatatccctttgttgggtttataccacttagcttgaaagaggttaaaacattacaattcattgttaagttgaatacagcaaaatgggagtcaaagttctgtttgccctgatctgcatcgctgtggccgaggccaagcccaccgagaacaacgaagacttcaacatcgtggccgtggccagcaacttcgcgaccacggatctcgatgctgaccgcgggaagttgcccggcaagaagctgccgctggaggtgctcaaagagatggaagccaatgcccggaaagctggctgcaccaggggctgtctgatctgcctgtcccacatcaagtgcacgcccaagatgaagaagttcatcccaggacgctgccacacctacgaaggcgacaaagagtccgcacagggcggcataggcgaggcgatcgtcgacattcctgagattcctgggttcaaggacttggagcccatggagcagttcatcgcacaggtcgatctgtgtgtggactgcacaactggctgcctcaaagggcttgccaacgtgcagtgttctgacctgctcaagaagtggctgccgcaacgctgtgcgacctttgccagcaagatccagggccaggtggacaagatcaagggggccggtggtgactaattaaaacagcctgtgggttgataaataattgtcaacccacaaagaaattctttaagtggatgctctcaaactcagggaaacctaaatctagttatagacaaggcaatcctgagccaagccgaagtagtaattagtaaggcctagtataccaaaccgcgatatctcttttctag

SEQ ID NO: 19 - RNA, 95 nt, synthetic construct
  source 1..95: mol_type = other RNA
ttaaaacagcggatgggtaccccaccatccgacccactgggtgtagtactctggtacttcgtacctttgtacgcctgttcttcccattgtaccct

SEQ ID NO: 20 - RNA, 95 nt, synthetic construct
  source 1..95: mol_type = other RNA
ttaaaacagcctgtgggttgttcccacccgcagggcccactgggcgctagcacactggtatcccggtacccttgtgcgcctgttttatataccct

SEQ ID NO: 21 - RNA, 96 nt, synthetic construct
  source 1..96: mol_type = other RNA
ttaaaacagctctggggttgctcccaccccagaggcccacgtggcggccagtactctggtattgcggtacctttgtacgcctgttttatactccct

SEQ ID NO: 22 - RNA, 93 nt, synthetic construct
  source 1..93: mol_type = other RNA
ttaaaatagctgctgggttgttcccatccagcaggcccactgggcgtgatactctggtattgcggtacctttgtatgcctattttacctccct

SEQ ID NO: 23 - RNA, 91 nt, synthetic construct
  source 1..91: mol_type = other RNA
ttaaaacagcctgggggttgtacccacccctggggcccacgcggcgccagtactctggtacgctagtacctttgtacgcctgttttcccca

SEQ ID NO: 24 - RNA, 626 nt, synthetic construct
  source 1..626: mol_type = other RNA
ttaaaacagcggatgggtaccccaccatccgacccactgggtgtagtactctggtacttcgtacctttgtacgcctgttcttcccattgtacccttcctgaacttccaacccaagtaacgttagaagctcaacatttagtacaacaggaagcaccacatccagtggtgtttagtacaagcacttctgtttccccggagcgaggtataggctgtacccactgccaaaaacctttaaccgttatccgccaaccaactacgtaaaagctagtagtattatgtttttaactaggcgttcgatcaggtggatttcccctccactagtttggtcgatgaggctaggaattccccacgggtgaccgtgtcctagcctgcgtggcggccaacccagcttatgctgggacgcctttttatagacatggtgtgaagactcgcatgtgcttggttgtgattcctccggcccctgaatgcggctaaccttaaccctggagccttgtgtcacaaaccagtgatgataaggtcgtaatgagcaattccgggacgggaccgactactttgggtgtccgtgtttcttatttttcttattattgtcttatggtcacagcatatatataacatatactgtgatc

SEQ ID NO: 25 - RNA, 743 nt, synthetic construct
  source 1..743: mol_type = other RNA
ttaaaacagcctgtgggttgttcccacccgcagggcccactgggcgctagcacactggtatcccggtacccttgtgcgcctgttttatataccctcccccttatgtaacttagaagtatgattcaaacggtcgacaggcggctcagtgcaccaactgagtcatgaccaagcacttctgttaccccggactgagtatcaataagctgttcacacggctgaaggagaaaacgttcgttacccggccaattacttcgagaaacctagtaccaccatgaaggttgcgcagtgtttcgctccacacaaccccagtgtagatcaggtcgatgagtcaccgcattccccacgggcgaccgtggcggtggctgcgttggcggcctgcccatggggcaacccatgggacgcttcaatactgacatggtgtgaagagtctattgagctaattggtagtcctccggcccctgaatgcggctaatcccaactgtggagcagatactcacaaaccagtgagcggtctgtcgtaacgggcaactccgcagcggaaccgactactttgggtgtccgtgtttctttttattcttacattggctgcttatggtgacaattgacaaattgttaccatatagctattggattggccatccggtgacaaacagagctattgtttacttgtttgttggtttcataccattaaattacaaggtcttagaaactctcaactttattttgacactcaatacagcaaa

SEQ ID NO: 26 - RNA, 747 nt, synthetic construct
  source 1..747: mol_type = other RNA
ttaaaacagctctggggttgctcccaccccagaggcccacgtggcggccagtactctggtattgcggtacctttgtacgcctgttttatactccctccccccgtgcaactttagaagaaatccacaaagttcaatagagggggtgcaaaccagcaccaccacgaacaagcacttctgtttccccggtgatgtcgtataagctgtacccacggctgaaggcgacggatccgttatccgcttgagtacttcgagaagcctagtattaccttggaatcttcgacgcgttgcgctcagcactctaccccgagtgtagcttaggtcgatgagtctgggcacgccccaccggcgacggtggcccaggctgcgttggcggcctacccatggctatcaccatgggacgctagttgtgaacaaggtgtgaagagcctattgagctacccaagagtcctccggcccctgaatgcggctaatcctaaccacggagcaagtgtcctcaacccaggggatggcttgtcgtaacgcgaaagtctgtggcggaaccgactactttgggtgtccgtgtttccttttatttttatgtatggctgcttatggtgacaatcaaaggttgttaccataaagcaatttggattggccatccggtgagaatcaaacatattatctacctgtttgttgggttttcttcttttacttgaacaatacctctaataataactgctatattgtcaataagacattatcatcaca

SEQ ID NO: 27 - RNA, 666 nt, synthetic construct
  source 1..666: mol_type = other RNA
ttaaaatagctgctgggttgttcccatccagcaggcccactgggcgtgatactctggtattgcggtacctttgtatgcctattttacctcccttccccctgaaacttagaagaaagaaacaaacacgctcactaggtacactgcatccagcagtgtaatgagcaagcacttctgtttccccggaagggatatatggtacgctgtgcaaacggcggaaattaatcctaccgttaaccgcccatctactccgagaagcctagtacctaattgaacttatcaatggagttgcgctcagcaggtgaccctgacctgccagctccggctgatggacctgggcatcccccacaggcgactgtggcccaggtcgcgtggcggccggcccactcttttgagtgggacgccttgataatgacaaggtgggaagagcctattgggctagctggtttcctccggcctcctgaatgcggctaaccctaaccccggagcatatggtggcaacccagccactggtatgtcgtaacgcgtaagtctgggatgggaccgactactttggagagtccgtgtttccattattttctttattgaatcttatggtgacaaattgggagttactcgggtgacgattgattattacttctgaaaacgtagagatatagaatcaacaca

SEQ ID NO: 28 - RNA, 812 nt, synthetic construct
  source 1..812: mol_type = other RNA
ttaaaacagcctgggggttgtacccacccctggggcccacgcggcgccagtactctggtacgctagtacctttgtacgcctgttttccccacccttaaataaattaagattaccactgctgtggggagtagtccgactccgcaccgatacgtcgcaccagtgaactggttcgcttagaacctttgcacggagcagctggtatccccccccgtaacttagaagcctggacaaaccgaccaatagaggcgttgtagccagcagcgcaacggtcaagcacttctgtttccccggcgccatgcgtcgttacccgcccggcctactgcgggaagcctagtaggaccccaatcggacgcgcggttgcgttcagccacaaccccagtggtagctctgaggaatgggactcgcctaccccccacagcaatgtggtggcttgtccgcgtgtgtcctcgggttcgctcgttgagcgatcaccgcaactctgagtaaggtctcaagagcctactgcgctaggtcggttctcctccggagccgtgaatgctgctaatcccaacctccgagcgtgtgcgcacaacccagtgttgctacgtcgtaatgcgtaagttggaggcggaacagactactttcggtactccgtgtttccttaatttttgttcattattacatggtgacattgactgacatttgtgaatttgcccgcctgcccttgaacatagctctctattacttgattgcatttcacaaaacaacccaactcactgttgaacttgttgacttcgcagtctacttgaacttacagtacaatcacattcaca

SEQ ID NO: 29 - RNA, 1500 nt, synthetic construct
  source 1..1500: mol_type = other RNA
gggtcacccgtcgcgcggtttggtatactaggccaacaatagatgacttacaactaatcggaaggtgcagagactcgacgggagctaccctaacgtcaagacgagggtaaagagagagtccaattctcaaagccaataggcagtagcgaaagctgcaagagaatgaccccaccatccgacccactgggtgtagtactctggtacttcgtacctttgtacgcctgttcttcccattgtacccttcctgaacttccaacccaagtaacgttagaagctcaacatttagtacaacaggaagcaccacatccagtggtgtttagtacaagcacttctgtttccccggagcgaggtataggctgtacccactgccaaaaacctttaaccgttatccgccaaccaactacgtaaaagctagtagtattatgtttttaactaggcgttcgatcaggtggatttcccctccactagtttggtcgatgaggctaggaattccccacgggtgaccgtgtcctagcctgcgtggcggccaacccagcttatgctgggacgcctttttatagacatggtgtgaagactcgcatgtgcttggttgtgattcctccggcccctgaatgcggctaaccttaaccctggagccttgtgtcacaaaccagtgatgataaggtcgtaatgagcaattccgggacgggaccgactactttgggtgtccgtgtttcttatttttcttattattgtcttatggtcacagcatatatataacatatactgtgatcatgggagtcaaagttctgtttgccctgatctgcatcgctgtggccgaggccaagcccaccgagaacaacgaagacttcaacatcgtggccgtggccagcaacttcgcgaccacggatctcgatgctgaccgcgggaagttgcccggcaagaagctgccgctggaggtgctcaaagagatggaagccaatgcccggaaagctggctgcaccaggggctgtctgatctgcctgtcccacatcaagtgcacgcccaagatgaagaagttcatcccaggacgctgccacacctacgaaggcgacaaagagtccgcacagggcggcataggcgaggcgatcgtcgacattcctgagattcctgggttcaaggacttggagcccatggagcagttcatcgcacaggtcgatctgtgtgtggactgcacaactggctgcctcaaagggcttgccaacgtgcagtgttctgacctgctcaagaagtggctgccgcaacgctgtgcgacctttgccagcaagatccagggccaggtggacaagatcaagggggccggtggtgactaattaaaacagcggatgggtaaataattgccccttaaagaagaaattctttaagtggatgctctcaaactcagggaaacctaaatctagttatagacaaggcaatcctgagccaagccgaagtagtaattagtaaggcctagtataccaaaccgcgatatctcttttctag

SEQ ID NO: 30 - RNA, 1617 nt, synthetic construct
  source 1..1617: mol_type = other RNA
gggtcacccgtcgcgcggtttggtatactaggccaacaatagatgacttacaactaatcggaaggtgcagagactcgacgggagctaccctaacgtcaagacgagggtaaagagagagtccaattctcaaagccaataggcagtagcgaaagctgcaagagaatgcccacccgcagggcccactgggcgctagcacactggtatcccggtacccttgtgcgcctgttttatataccctcccccttatgtaacttagaagtatgattcaaacggtcgacaggcggctcagtgcaccaactgagtcatgaccaagcacttctgttaccccggactgagtatcaataagctgttcacacggctgaaggagaaaacgttcgttacccggccaattacttcgagaaacctagtaccaccatgaaggttgcgcagtgtttcgctccacacaaccccagtgtagatcaggtcgatgagtcaccgcattccccacgggcgaccgtggcggtggctgcgttggcggcctgcccatggggcaacccatgggacgcttcaatactgacatggtgtgaagagtctattgagctaattggtagtcctccggcccctgaatgcggctaatcccaactgtggagcagatactcacaaaccagtgagcggtctgtcgtaacgggcaactccgcagcggaaccgactactttgggtgtccgtgtttctttttattcttacattggctgcttatggtgacaattgacaaattgttaccatatagctattggattggccatccggtgacaaacagagctattgtttacttgtttgttggtttcataccattaaattacaaggtcttagaaactctcaactttattttgacactcaatacagcaaaatgggagtcaaagttctgtttgccctgatctgcatcgctgtggccgaggccaagcccaccgagaacaacgaagacttcaacatcgtggccgtggccagcaacttcgcgaccacggatctcgatgctgaccgcgggaagttgcccggcaagaagctgccgctggaggtgctcaaagagatggaagccaatgcccggaaagctggctgcaccaggggctgtctgatctgcctgtcccacatcaagtgcacgcccaagatgaagaagttcatcccaggacgctgccacacctacgaaggcgacaaagagtccgcacagggcggcataggcgaggcgatcgtcgacattcctgagattcctgggttcaaggacttggagcccatggagcagttcatcgcacaggtcgatctgtgtgtggactgcacaactggctgcctcaaagggcttgccaacgtgcagtgttctgacctgctcaagaagtggctgccgcaacgctgtgcgacctttgccagcaagatccagggccaggtggacaagatcaagggggccggtggtgactaattaaaacagcctgtgggttgttaaataattgacccttaaagaagaaattctttaagtggatgctctcaaactcagggaaacctaaatctagttatagacaaggcaatcctgagccaagccgaagtagtaattagtaaggcctagtataccaaaccgcgatatctcttttctag

SEQ ID NO: 31 - RNA, 1621 nt, synthetic construct
  source 1..1621: mol_type = other RNA
gggtcacccgtcgcgcggtttggtatactaggccaacaatagatgacttacaactaatcggaaggtgcagagactcgacgggagctaccctaacgtcaagacgagggtaaagagagagtccaattctcaaagccaataggcagtagcgaaagctgcaagagaatgcccaccccagaggcccacgtggcggccagtactctggtattgcggtacctttgtacgcctgttttatactccctccccccgtgcaactttagaagaaatccacaaagttcaatagagggggtgcaaaccagcaccaccacgaacaagcacttctgtttccccggtgatgtcgtataagctgtacccacggctgaaggcgacggatccgttatccgcttgagtacttcgagaagcctagtattaccttggaatcttcgacgcgttgcgctcagcactctaccccgagtgtagcttaggtcgatgagtctgggcacgccccaccggcgacggtggcccaggctgcgttggcggcctacccatggctatcaccatgggacgctagttgtgaacaaggtgtgaagagcctattgagctacccaagagtcctccggcccctgaatgcggctaatcctaaccacggagcaagtgtcctcaacccaggggatggcttgtcgtaacgcgaaagtctgtggcggaaccgactactttgggtgtccgtgtttccttttatttttatgtatggctgcttatggtgacaatcaaaggttgttaccataaagcaatttggattggccatccggtgagaatcaaacatattatctacctgtttgttgggttttcttcttttacttgaacaatacctctaataataactgctatattgtcaataagacattatcatcacaatgggagtcaaagttctgtttgccctgatctgcatcgctgtggccgaggccaagcccaccgagaacaacgaagacttcaacatcgtggccgtggccagcaacttcgcgaccacggatctcgatgctgaccgcgggaagttgcccggcaagaagctgccgctggaggtgctcaaagagatggaagccaatgcccggaaagctggctgcaccaggggctgtctgatctgcctgtcccacatcaagtgcacgcccaagatgaagaagttcatcccaggacgctgccacacctacgaaggcgacaaagagtccgcacagggcggcataggcgaggcgatcgtcgacattcctgagattcctgggttcaaggacttggagcccatggagcagttcatcgcacaggtcgatctgtgtgtggactgcacaactggctgcctcaaagggcttgccaacgtgcagtgttctgacctgctcaagaagtggctgccgcaacgctgtgcgacctttgccagcaagatccagggccaggtggacaagatcaagggggccggtggtgactaattaaaacagctctggggttgctaaataattggcccttaaagaagaaattctttaagtggatgctctcaaactcagggaaacctaaatctagttatagacaaggcaatcctgagccaagccgaagtagtaattagtaaggcctagtataccaaaccgcgatatctcttttctag

SEQ ID NO: 32 - RNA, 1540 nt, synthetic construct
  source 1..1540: mol_type = other RNA
gggtcacccgtcgcgcggtttggtatactaggccaacaatagatgacttacaactaatcggaaggtgcagagactcgacgggagctaccctaacgtcaagacgagggtaaagagagagtccaattctcaaagccaataggcagtagcgaaagctgcaagagaatgcccatccagcaggcccactgggcgtgatactctggtattgcggtacctttgtatgcctattttacctcccttccccctgaaacttagaagaaagaaacaaacacgctcactaggtacactgcatccagcagtgtaatgagcaagcacttctgtttccccggaagggatatatggtacgctgtgcaaacggcggaaattaatcctaccgttaaccgcccatctactccgagaagcctagtacctaattgaacttatcaatggagttgcgctcagcaggtgaccctgacctgccagctccggctgatggacctgggcatcccccacaggcgactgtggcccaggtcgcgtggcggccggcccactcttttgagtgggacgccttgataatgacaaggtgggaagagcctattgggctagctggtttcctccggcctcctgaatgcggctaaccctaaccccggagcatatggtggcaacccagccactggtatgtcgtaacgcgtaagtctgggatgggaccgactactttggagagtccgtgtttccattattttctttattgaatcttatggtgacaaattgggagttactcgggtgacgattgattattacttctgaaaacgtagagatatagaatcaacacaatgggagtcaaagttctgtttgccctgatctgcatcgctgtggccgaggccaagcccaccgagaacaacgaagacttcaacatcgtggccgtggccagcaacttcgcgaccacggatctcgatgctgaccgcgggaagttgcccggcaagaagctgccgctggaggtgctcaaagagatggaagccaatgcccggaaagctggctgcaccaggggctgtctgatctgcctgtcccacatcaagtgcacgcccaagatgaagaagttcatcccaggacgctgccacacctacgaaggcgacaaagagtccgcacagggcggcataggcgaggcgatcgtcgacattcctgagattcctgggttcaaggacttggagcccatggagcagttcatcgcacaggtcgatctgtgtgtggactgcacaactggctgcctcaaagggcttgccaacgtgcagtgttctgacctgctcaagaagtggctgccgcaacgctgtgcgacctttgccagcaagatccagggccaggtggacaagatcaagggggccggtggtgactaattaaaatagctgctgggttgttaaataattgacccttaaagaagaaattctttaagtggatgctctcaaactcagggaaacctaaatctagttatagacaaggcaatcctgagccaagccgaagtagtaattagtaaggcctagtataccaaaccgcgatatctcttttctag

SEQ ID NO: 33 - RNA, 1686 nt, synthetic construct
  source 1..1686: mol_type = other RNA
gggtcacccgtcgcgcggtttggtatactaggccaacaatagatgacttacaactaatcggaaggtgcagagactcgacgggagctaccctaacgtcaagacgagggtaaagagagagtccaattctcaaagccaataggcagtagcgaaagctgcaagagaatgacccacccctggggcccacgcggcgccagtactctggtacgctagtacctttgtacgcctgttttccccacccttaaataaattaagattaccactgctgtggggagtagtccgactccgcaccgatacgtcgcaccagtgaactggttcgcttagaacctttgcacggagcagctggtatccccccccgtaacttagaagcctggacaaaccgaccaatagaggcgttgtagccagcagcgcaacggtcaagcacttctgtttccccggcgccatgcgtcgttacccgcccggcctactgcgggaagcctagtaggaccccaatcggacgcgcggttgcgttcagccacaaccccagtggtagctctgaggaatgggactcgcctaccccccacagcaatgtggtggcttgtccgcgtgtgtcctcgggttcgctcgttgagcgatcaccgcaactctgagtaaggtctcaagagcctactgcgctaggtcggttctcctccggagccgtgaatgctgctaatcccaacctccgagcgtgtgcgcacaacccagtgttgctacgtcgtaatgcgtaagttggaggcggaacagactactttcggtactccgtgtttccttaatttttgttcattattacatggtgacattgactgacatttgtgaatttgcccgcctgcccttgaacatagctctctattacttgattgcatttcacaaaacaacccaactcactgttgaacttgttgacttcgcagtctacttgaacttacagtacaatcacattcacaatgggagtcaaagttctgtttgccctgatctgcatcgctgtggccgaggccaagcccaccgagaacaacgaagacttcaacatcgtggccgtggccagcaacttcgcgaccacggatctcgatgctgaccgcgggaagttgcccggcaagaagctgccgctggaggtgctcaaagagatggaagccaatgcccggaaagctggctgcaccaggggctgtctgatctgcctgtcccacatcaagtgcacgcccaagatgaagaagttcatcccaggacgctgccacacctacgaaggcgacaaagagtccgcacagggcggcataggcgaggcgatcgtcgacattcctgagattcctgggttcaaggacttggagcccatggagcagttcatcgcacaggtcgatctgtgtgtggactgcacaactggctgcctcaaagggcttgccaacgtgcagtgttctgacctgctcaagaagtggctgccgcaacgctgtgcgacctttgccagcaagatccagggccaggtggacaagatcaagggggccggtggtgactaattaaaacagcctgggggttgtaaataattgcaccttaaagaagaaattctttaagtggatgctctcaaactcagggaaacctaaatctagttatagacaaggcaatcctgagccaagccgaagtagtaattagtaaggcctagtataccaaaccgcgatatctcttttctag

SEQ ID NO: 34 - RNA, 587 nt, synthetic construct
  source 1..587: mol_type = other RNA
cccctctccctcccccccccctaacgttactggccgaagccgcttggaataaggccggtgtgcgtttgtctatatgttattttccaccatattgccgtcttttggcaatgtgagggcccggaaacctggccctgtcttcttgacgagcattcctaggggtctttcccctctcgccaaaggaatgcaaggtctgttgaatgtcgtgaaggaagcagttcctctggaagcttcttgaagacaaacaacgtctgtagcgaccctttgcaggcagcggaaccccccacctggcgacaggtgcctctgcggccaaaagccacgtgtataagatacacctgcaaaggcggcacaaccccagtgccacgttgtgagttggatagttgtggaaagagtcaaatggctctcctcaagcgtattcaacaaggggctgaaggatgcccagaaggtaccccattgtatgggatctgatctggggcctcggtacacatgctttacatgtgtttagtcgaggttaaaaaaacgtctaggccccccgaaccacggggacgtggttttcctttgaaaaacacgatgataatatggccacaacc

SEQ ID NO: 35 - RNA, 223 nt, synthetic construct
  source 1..223: mol_type = other RNA
agtacccttcaccaaagcaaaaatgtgatcttgcttgtaaatacaattttgagaggttaataaattacaagtagtgctatttttgtatttaggttagctatttagctttacgttccaggatgcctagtggcagccccacaatatccaggaagccctctctgcggtttttcagattaggtagtcgaaaaacctaagaaatttacctgctacatttcaagatacc

SEQ ID NO: 36 - RNA, 676 nt, synthetic construct
  source 1..676: mol_type = other RNA
ttaaaacagcctgtgggttgatcccacccacaggcccattgggcgctagcactctggtatcacggtacctttgtgcgcctgttttataccccctctccctcccccccccctaacgttactggccgaagccgcttggaataaggccggtgtgcgtttgtctatatgttattttccaccatattgccgtcttttggcaatgtgagggcccggaaacctggccctgtcttcttgacgagcattcctaggggtctttcccctctcgccaaaggaatgcaaggtctgttgaatgtcgtgaaggaagcagttcctctggaagcttcttgaagacaaacaacgtctgtagcgaccctttgcaggcagcggaaccccccacctggcgacaggtgcctctgcggccaaaagccacgtgtataagatacacctgcaaaggcggcacaaccccagtgccacgttgtgagttggatagttgtggaaagagtcaaatggctctcctcaagcgtattcaacaaggggctgaaggatgcccagaaggtaccccattgtatgggatctgatctggggcctcggtgcacatgctttacatgtgtttagtcgaggttaaaaaaacgtctaggccccccgaaccacggggacgtggttttcctttgaaaaacacgatgataatatggccacaacc

SEQ ID NO: 37 - RNA, 317 nt, synthetic construct
  source 1..317: mol_type = other RNA
ttaaaacagcctgtgggttgatcccacccacaggcccattgggcgctagcactctggtatcacggtacctttgtgcgcctgttttataccccctagtacccttcaccaaagcaaaaatgtgatcttgcttgtaaatacaattttgagaggttaataaattacaagtagtgctatttttgtatttaggttagctatttagctttacgttccaggatgcctagtggcagccccacaatatccaggaagccctctctgcggtttttcagattaggtagtcgaaaaacctaagaaatttacctgctacatttcaagatacc

SEQ ID NO: 38 - RNA, 1234 nt, synthetic construct
  source 1..1234: mol_type = other RNA
ttaaaacagcctgtgggttgatcccacccacaggcccattgggcgctagcactctggtatcacggtacctttgtgcgcctgttttataccccctctccctcccccccccctaacgttactggccgaagccgcttggaataaggccggtgtgcgtttgtctatatgttattttccaccatattgccgtcttttggcaatgtgagggcccggaaacctggccctgtcttcttgacgagcattcctaggggtctttcccctctcgccaaaggaatgcaaggtctgttgaatgtcgtgaaggaagcagttcctctggaagcttcttgaagacaaacaacgtctgtagcgaccctttgcaggcagcggaaccccccacctggcgacaggtgcctctgcggccaaaagccacgtgtataagatacacctgcaaaggcggcacaaccccagtgccacgttgtgagttggatagttgtggaaagagtcaaatggctctcctcaagcgtattcaacaaggggctgaaggatgcccagaaggtaccccattgtatgggatctgatctggggcctcggtgcacatgctttacatgtgtttagtcgaggttaaaaaaacgtctaggccccccgaaccacggggacgtggttttcctttgaaaaacacgatgataatatggccacaaccatgggagtcaaagttctgtttgccctgatctgcatcgctgtggccgaggccaagcccaccgagaacaacgaagacttcaacatcgtggccgtggccagcaacttcgcgaccacggatctcgatgctgaccgcgggaagttgcccggcaagaagctgccgctggaggtgctcaaagagatggaagccaatgcccggaaagctggctgcaccaggggctgtctgatctgcctgtcccacatcaagtgcacgcccaagatgaagaagttcatcccaggacgctgccacacctacgaaggcgacaaagagtccgcacagggcggcataggcgaggcgatcgtcgacattcctgagattcctgggttcaaggacttggagcccatggagcagttcatcgcacaggtcgatctgtgtgtggactgcacaactggctgcctcaaagggcttgccaacgtgcagtgttctgacctgctcaagaagtggctgccgcaacgctgtgcgacctttgccagcaagatccagggccaggtggacaagatcaagggggccggtggtgactaa

SEQ ID NO: 39 - RNA, 875 nt, synthetic construct
  source 1..875: mol_type = other RNA
ttaaaacagcctgtgggttgatcccacccacaggcccattgggcgctagcactctggtatcacggtacctttgtgcgcctgttttataccccctagtacccttcaccaaagcaaaaatgtgatcttgcttgtaaatacaattttgagaggttaataaattacaagtagtgctatttttgtatttaggttagctatttagctttacgttccaggatgcctagtggcagccccacaatatccaggaagccctctctgcggtttttcagattaggtagtcgaaaaacctaagaaatttacctgctacatttcaagataccatgggagtcaaagttctgtttgccctgatctgcatcgctgtggccgaggccaagcccaccgagaacaacgaagacttcaacatcgtggccgtggccagcaacttcgcgaccacggatctcgatgctgaccgcgggaagttgcccggcaagaagctgccgctggaggtgctcaaagagatggaagccaatgcccggaaagctggctgcaccaggggctgtctgatctgcctgtcccacatcaagtgcacgcccaagatgaagaagttcatcccaggacgctgccacacctacgaaggcgacaaagagtccgcacagggcggcataggcgaggcgatcgtcgacattcctgagattcctgggttcaaggacttggagcccatggagcagttcatcgcacaggtcgatctgtgtgtggactgcacaactggctgcctcaaagggcttgccaacgtgcagtgttctgacctgctcaagaagtggctgccgcaacgctgtgcgacctttgccagcaagatccagggccaggtggacaagatcaagggggccggtggtgactaa

SEQ ID NO: 40 - RNA, 1550 nt, synthetic construct
  source 1..1550: mol_type = other RNA
gggtcacccgtcgcgcggtttggtatactaggccaacaatagatgacttacaactaatcggaaggtgcagagactcgacgggagctaccctaacgtcaagacgagggtaaagagagagtccaattctcaaagccaataggcagtagcgaaagctgcaagagaatgcccacccacaggcccattgggcgctagcactctggtatcacggtacctttgtgcgcctgttttataccccctctccctcccccccccctaacgttactggccgaagccgcttggaataaggccggtgtgcgtttgtctatatgttattttccaccatattgccgtcttttggcaatgtgagggcccggaaacctggccctgtcttcttgacgagcattcctaggggtctttcccctctcgccaaaggaatgcaaggtctgttgaatgtcgtgaaggaagcagttcctctggaagcttcttgaagacaaacaacgtctgtagcgaccctttgcaggcagcggaaccccccacctggcgacaggtgcctctgcggccaaaagccacgtgtataagatacacctgcaaaggcggcacaaccccagtgccacgttgtgagttggatagttgtggaaagagtcaaatggctctcctcaagcgtattcaacaaggggctgaaggatgcccagaaggtaccccattgtatgggatctgatctggggcctcggtgcacatgctttacatgtgtttagtcgaggttaaaaaaacgtctaggccccccgaaccacggggacgtggttttcctttgaaaaacacgatgataatatggccacaaccatgggagtcaaagttctgtttgccctgatctgcatcgctgtggccgaggccaagcccaccgagaacaacgaagacttcaacatcgtggccgtggccagcaacttcgcgaccacggatctcgatgctgaccgcgggaagttgcccggcaagaagctgccgctggaggtgctcaaagagatggaagccaatgcccggaaagctggctgcaccaggggctgtctgatctgcctgtcccacatcaagtgcacgcccaagatgaagaagttcatcccaggacgctgccacacctacgaaggcgacaaagagtccgcacagggcggcataggcgaggcgatcgtcgacattcctgagattcctgggttcaaggacttggagcccatggagcagttcatcgcacaggtcgatctgtgtgtggactgcacaactggctgcctcaaagggcttgccaacgtgcagtgttctgacctgctcaagaagtggctgccgcaacgctgtgcgacctttgccagcaagatccagggccaggtggacaagatcaagggggccggtggtgactaattaaaacagcctgtgggttgataaataattgtcccttaaagaagaaattctttaagtggatgctctcaaactcagggaaacctaaatctagttatagacaaggcaatcctgagccaagccgaagtagtaattagtaaggcctagtataccaaaccgcgatatctcttttctag

SEQ ID NO: 41 - RNA, 1191 nt, synthetic construct
  source 1..1191: mol_type = other RNA
gggtcacccgtcgcgcggtttggtatactaggccaacaatagatgacttacaactaatcggaaggtgcagagactcgacgggagctaccctaacgtcaagacgagggtaaagagagagtccaattctcaaagccaataggcagtagcgaaagctgcaagagaatgcccacccacaggcccattgggcgctagcactctggtatcacggtacctttgtgcgcctgttttataccccctagtacccttcaccaaagcaaaaatgtgatcttgcttgtaaatacaattttgagaggttaataaattacaagtagtgctatttttgtatttaggttagctatttagctttacgttccaggatgcctagtggcagccccacaatatccaggaagccctctctgcggtttttcagattaggtagtcgaaaaacctaagaaatttacctgctacatttcaagataccatgggagtcaaagttctgtttgccctgatctgcatcgctgtggccgaggccaagcccaccgagaacaacgaagacttcaacatcgtggccgtggccagcaacttcgcgaccacggatctcgatgctgaccgcgggaagttgcccggcaagaagctgccgctggaggtgctcaaagagatggaagccaatgcccggaaagctggctgcaccaggggctgtctgatctgcctgtcccacatcaagtgcacgcccaagatgaagaagttcatcccaggacgctgccacacctacgaaggcgacaaagagtccgcacagggcggcataggcgaggcgatcgtcgacattcctgagattcctgggttcaaggacttggagcccatggagcagttcatcgcacaggtcgatctgtgtgtggactgcacaactggctgcctcaaagggcttgccaacgtgcagtgttctgacctgctcaagaagtggctgccgcaacgctgtgcgacctttgccagcaagatccagggccaggtggacaagatcaagggggccggtggtgactaattaaaacagcctgtgggttgataaataattgtcccttaaagaagaaattctttaagtggatgctctcaaactcagggaaacctaaatctagttatagacaaggcaatcctgagccaagccgaagtagtaattagtaaggcctagtataccaaaccgcgatatctcttttctag

SEQ ID NO: 42 - RNA, 1636 nt, synthetic construct
  source 1..1636: mol_type = other RNA
gggagaccctcgaccgtcgattgtccactggtcaacaatagatgacttacaactaatcggaaggtgcagagactcgacgggagctaccctaacgtcaagacgagggtaaagagagagtccaattctcaaagccaataggcagtagcgaaagctgcaagagaatgaaaatccgttgaccttaaacggtcgtgtgggttcaagtccctccacccccacgccggaaacgcaatagccgaaaaacaaaaaacaaaaaaaacaaaaaaaaaaccaaaaaaacaaaacacacccctctccctcccccccccctaacgttactggccgaagccgcttggaataaggccggtgtgcgtttgtctatatgttattttccaccatattgccgtcttttggcaatgtgagggcccggaaacctggccctgtcttcttgacgagcattcctaggggtctttcccctctcgccaaaggaatgcaaggtctgttgaatgtcgtgaaggaagcagttcctctggaagcttcttgaagacaaacaacgtctgtagcgaccctttgcaggcagcggaaccccccacctggcgacaggtgcctctgcggccaaaagccacgtgtataagatacacctgcaaaggcggcacaaccccagtgccacgttgtgagttggatagttgtggaaagagtcaaatggctctcctcaagcgtattcaacaaggggctgaaggatgcccagaaggtaccccattgtatgggatctgatctggggcctcggtacacatgctttacatgtgtttagtcgaggttaaaaaaacgtctaggccccccgaaccacggggacgtggttttcctttgaaaaacacgatgataatatggccacaaccatgggagtcaaagttctgtttgccctgatctgcatcgctgtggccgaggccaagcccaccgagaacaacgaagacttcaacatcgtggccgtggccagcaacttcgcgaccacggatctcgatgctgaccgcgggaagttgcccggcaagaagctgccgctggaggtgctcaaagagatggaagccaatgcccggaaagctggctgcaccaggggctgtctgatctgcctgtcccacatcaagtgcacgcccaagatgaagaagttcatcccaggacgctgccacacctacgaaggcgacaaagagtccgcacagggcggcataggcgaggcgatcgtcgacattcctgagattcctgggttcaaggacttggagcccatggagcagttcatcgcacaggtcgatctgtgtgtggactgcacaactggctgcctcaaagggcttgccaacgtgcagtgttctgacctgctcaagaagtggctgccgcaacgctgtgcgacctttgccagcaagatccagggccaggtggacaagatcaagggggccggtggtgactaaaaaaaacaaaaaacaaaacggctattatgcgttaccggcgagacgctacggacttaaataattgagccttaaagaagaaattctttaagtggatgctctcaaactcagggaaacctaaatctagttatagacaaggcaatcctgagccaagccgaagtagtaattagtaagaccagtggacaatcgacggataacagcatatctag

SEQ ID NO: 43 - RNA, 1272 nt, synthetic construct
  source 1..1272: mol_type = other RNA
gggagaccctcgaccgtcgattgtccactggtcaacaatagatgacttacaactaatcggaaggtgcagagactcgacgggagctaccctaacgtcaagacgagggtaaagagagagtccaattctcaaagccaataggcagtagcgaaagctgcaagagaatgaaaatccgttgaccttaaacggtcgtgtgggttcaagtccctccacccccacgccggaaacgcaatagccgaaaaacaaaaaacaaaaaaaacaaaaaaaaaaccaaaaaaacaaaacacaagtacccttcaccaaagcaaaaatgtgatcttgcttgtaaatacaattttgagaggttaataaattacaagtagtgctatttttgtatttaggttagctatttagctttacgttccaggatgcctagtggcagccccacaatatccaggaagccctctctgcggtttttcagattaggtagtcgaaaaacctaagaaatttacctgctacatttcaagataccatgggagtcaaagttctgtttgccctgatctgcatcgctgtggccgaggccaagcccaccgagaacaacgaagacttcaacatcgtggccgtggccagcaacttcgcgaccacggatctcgatgctgaccgcgggaagttgcccggcaagaagctgccgctggaggtgctcaaagagatggaagccaatgcccggaaagctggctgcaccaggggctgtctgatctgcctgtcccacatcaagtgcacgcccaagatgaagaagttcatcccaggacgctgccacacctacgaaggcgacaaagagtccgcacagggcggcataggcgaggcgatcgtcgacattcctgagattcctgggttcaaggacttggagcccatggagcagttcatcgcacaggtcgatctgtgtgtggactgcacaactggctgcctcaaagggcttgccaacgtgcagtgttctgacctgctcaagaagtggctgccgcaacgctgtgcgacctttgccagcaagatccagggccaggtggacaagatcaagggggccggtggtgactaaaaaaaacaaaaaacaaaacggctattatgcgttaccggcgagacgctacggacttaaataattgagccttaaagaagaaattctttaagtggatgctctcaaactcagggaaacctaaatctagttatagacaaggcaatcctgagccaagccgaagtagtaattagtaagaccagtggacaatcgacggataacagcatatctag

SEQ ID NO: 44 - DNA, 22 bp, synthetic construct
  source 1..22: mol_type = other DNA
gtctcctctgacttcaacagcg

SEQ ID NO: 45 - DNA, 22 bp, synthetic construct
  source 1..22: mol_type = other DNA
accaccctgttgctgtagccaa

SEQ ID NO: 46 - DNA, 22 bp, synthetic construct
  source 1..22: mol_type = other DNA
agacagccactcacctcttcag

SEQ ID NO: 47 - DNA, 22 bp, synthetic construct
  source 1..22: mol_type = other DNA
ttctgccagtgcctctttgctg

SEQ ID NO: 48 - DNA, 22 bp, synthetic construct
  source 1..22: mol_type = other DNA
cacctcagttgctgatgaaggc

SEQ ID NO: 49 - DNA, 23 bp, synthetic construct
  source 1..23: mol_type = other DNA
gtcagaaggaagcacttgctacc

SEQ ID NO: 50 - DNA, 22 bp, synthetic construct
  source 1..22: mol_type = other DNA
cctgctgctttgcctacattgc

SEQ ID NO: 51 - DNA, 22 bp, synthetic construct
  source 1..22: mol_type = other DNA
acacacttggcggttctttcgg

SEQ ID NO: 52 - DNA, 24 bp, synthetic construct
  source 1..24: mol_type = other DNA
cttggattcctacaaagaagcagc

SEQ ID NO: 53 - DNA, 22 bp, synthetic construct
  source 1..22: mol_type = other DNA
tcctccttctggaactgctgca

SEQ ID NO: 54 - RNA, 1790 nt, synthetic construct
  source 1..1790: mol_type = other RNA
gggagaccctcgaccgtcgattgtccactggtcaacaatagatgacttacaactaatcggaaggtgcagagactcgacgggagctaccctaacgtcaagacgagggtaaagagagagtccaattctcaaagccaataggcagtagcgaaagctgcaagagaatgaaaatccgttgaccttaaacggtcgtgtgggttcaagtccctccacccccacgccggaaacgcaatagccgaaaaacaaaaaacaaaaaaaacaaaaaaaaaaccaaaaaaacaaaacacattaaaacagcctgtgggttgatcccacccacaggcccattgggcgctagcactctggtatcacggtacctttgtgcgcctgttttataccccctcccccaactgtaacttagaagtaacacacaccgatcaacagtcagcgtggcacaccagccacgttttgatcaagcacttctgttaccccggactgagtatcaatagactgctcacgcggttgaaggagaaagcgttcgttatccggccaactacttcgaaaaacctagtaacaccgtggaagttgcagagtgtttcgctcagcactaccccagtgtagatcaggtcgatgagtcaccgcattccccacgggcgaccgtggcggtggctgcgttggcggcctgcccatggggaaacccatgggacgctctaatacagacatggtgcgaagagtctattgagctagttggtagtcctccggcccctgaatgcggctaatcctaactgcggagcacacaccctcaagccagagggcagtgtgtcgtaacgggcaactctgcagcggaaccgactactttgggtgtccgtgtttcattttattcctatactggctgcttatggtgacaattgagagatcgttaccatatagctattggattggccatccggtgactaatagagctattatatatccctttgttgggtttataccacttagcttgaaagaggttaaaacattacaattcattgttaagttgaatacagcaaaatgggagtcaaagttctgtttgccctgatctgcatcgctgtggccgaggccaagcccaccgagaacaacgaagacttcaacatcgtggccgtggccagcaacttcgcgaccacggatctcgatgctgaccgcgggaagttgcccggcaagaagctgccgctggaggtgctcaaagagatggaagccaatgcccggaaagctggctgcaccaggggctgtctgatctgcctgtcccacatcaagtgcacgcccaagatgaagaagttcatcccaggacgctgccacacctacgaaggcgacaaagagtccgcacagggcggcataggcgaggcgatcgtcgacattcctgagattcctgggttcaaggacttggagcccatggagcagttcatcgcacaggtcgatctgtgtgtggactgcacaactggctgcctcaaagggcttgccaacgtgcagtgttctgacctgctcaagaagtggctgccgcaacgctgtgcgacctttgccagcaagatccagggccaggtggacaagatcaagggggccggtggtgactaaaaaaaacaaaaaacaaaacggctattatgcgttaccggcgagacgctacggacttaaataattgagccttaaagaagaaattctttaagtggatgctctcaaactcagggaaacctaaatctagttatagacaaggcaatcctgagccaagccgaagtagtaattagtaagaccagtggacaatcgacggataacagcatatctag

SEQ ID NO: 55 - RNA, 1617 nt, synthetic construct
  source 1..1617: mol_type = other RNA
gggtcacccgtcgcgcggtttggtatactaggccaacaatagatgacttacaactaatcggaaggtgcagagactcgacgggagctaccctaacgtcaagacgagggtaaagagagagtccaattctcaaagccaataggcagtagcgaaagctgcaagagaatgcccacccacagggcccactgggcgttagcacactggtatcacggtacctttgtgcgcctgttttatactcccccccctaaggaaactttagaagcaaagcaattgtgatcaatagtgggtatggcacaccagtcatatcttgatcaagcacttctgttcccccggacttagtaccaatagactgctcaagcggttgaaggggaaaacgttcgttatccggccaactacttcgagaaacctagtagcaccatgaaagttgcggagtgtttcgctcagcacttcccccgtgtagatcaggctgatgagtcaccgtattccccacgggcgaccgtgacggtggctgcgttggcggcctgcccatggggtaacccatgggacgctctaaaacagacacggtgcgaagagtctattgagctagttggtagtcctccggcccctgaatgcggccaatcctaactgcggagcacatactcccaatccagggagcagtgtgtcgtaatgggtaactctgcagcggaaccgactactttgggtgtccgtgtttccttttattctcacattgactgcttatggtgacaattgaaagattgttaccatatagctattggattggtcatccggtgagcaatagagctattgtttatcaatttgttggatttgtaccactcaacttttctgttttgagaacactcaactacatcttactgctaaacacatcaaaatgggagtcaaagttctgtttgccctgatctgcatcgctgtggccgaggccaagcccaccgagaacaacgaagacttcaacatcgtggccgtggccagcaacttcgcgaccacggatctcgatgctgaccgcgggaagttgcccggcaagaagctgccgctggaggtgctcaaagagatggaagccaatgcccggaaagctggctgcaccaggggctgtctgatctgcctgtcccacatcaagtgcacgcccaagatgaagaagttcatcccaggacgctgccacacctacgaaggcgacaaagagtccgcacagggcggcataggcgaggcgatcgtcgacattcctgagattcctgggttcaaggacttggagcccatggagcagttcatcgcacaggtcgatctgtgtgtggactgcacaactggctgcctcaaagggcttgccaacgtgcagtgttctgacctgctcaagaagtggctgccgcaacgctgtgcgacctttgccagcaagatccagggccaggtggacaagatcaagggggccggtggtgactaattaaaacagcctgtgggttgttaaataattgacccttaaagaagaaattctttaagtggatgctctcaaactcagggaaacctaaatctagttatagacaaggcaatcctgagccaagccgaagtagtaattagtaaggcctagtataccaaaccgcgatatctcttttctag

SEQ ID NO: 56 - RNA, 1618 nt, synthetic construct
  source 1..1618: mol_type = other RNA
gggtcacccgtcgcgcggtttggtatactaggccaacaatagatgacttacaactaatcggaaggtgcagagactcgacgggagctaccctaacgtcaagacgagggtaaagagagagtccaattctcaaagccaataggcagtagcgaaagctgcaagagaatgacccaccccagaggcccacgtggcggctagtactccggtattacggtacccttgtacgcctgttttatactccctccctcgtaacttagaagcacaaaaccaagttcaatagaagggggtgcaaaccagtaccaccacgaacaagcatttctgtttccccggtgatgttgtatagactgcccgcgcggttgaaagcaacggatccgttacccgctcaagtacttcgagaagcctagtattaccttggaatcttcgatgcgttgcgttcagcactcgaccctggagtgtagcttaggctgatgagtctggacgtccctcaccggtgacggtggtccaggctgcgttggcggcctacctatggctaacgccataggacgctagttgtgaacaaggtgtgaagagcctattgagctacttgagagtcctccggcccctgaatgcggctaatcctaaccatggagcaggcggtcacagaccagtgactagcttgtcgtaatgcgcaagtctatggcggaaccgactactttgggtgtccgtgtttccttttatttttattatggctgcttatggtgacaatcattgattgttatcataaagcgaattggattggccatccggtgaaagcgagacttactatttacttacttgttggacttaccacacttaatacatttattctaggtgtcacttgtatagcaattagaatcaaacagttgcatcataatgggagtcaaagttctgtttgccctgatctgcatcgctgtggccgaggccaagcccaccgagaacaacgaagacttcaacatcgtggccgtggccagcaacttcgcgaccacggatctcgatgctgaccgcgggaagttgcccggcaagaagctgccgctggaggtgctcaaagagatggaagccaatgcccggaaagctggctgcaccaggggctgtctgatctgcctgtcccacatcaagtgcacgcccaagatgaagaagttcatcccaggacgctgccacacctacgaaggcgacaaagagtccgcacagggcggcataggcgaggcgatcgtcgacattcctgagattcctgggttcaaggacttggagcccatggagcagttcatcgcacaggtcgatctgtgtgtggactgcacaactggctgcctcaaagggcttgccaacgtgcagtgttctgacctgctcaagaagtggctgccgcaacgctgtgcgacctttgccagcaagatccagggccaggtggacaagatcaagggggccggtggtgactaattaaaacagctctggggttgtaaataattgcaccttaaagaagaaattctttaagtggatgctctcaaactcagggaaacctaaatctagttatagacaaggcaatcctgagccaagccgaagtagtaattagtaaggcctagtataccaaaccgcgatatctcttttctag

SEQ ID NO: 57 - RNA, 1777 nt, synthetic construct
  source 1..1777: mol_type = other RNA
gggtcacccgtcgcgcggtttggtatactaggccaacaatagatgacttacaactaatcggaaggtgcagagactcgacgggagctaccctaacgtcaagacgagggtaaagagagagtccaattctcaaagccaataggcagtagcgaaagctgcaagagaatgcccacccacaggcccattgggcgctagcactctggtatcacggtacctttgtgcgcctgttttataccccctcccccaactgtaacttagaagtaacacacaccgatcaacagtcagcgtggcacaccagccacgttttgatcaagcacttctgttaccccggactgagtatcaatagactgctcacgcggttgaaggagaaagcgttcgttatccggccaactacttcgaaaaacctagtaacaccgtggaagttgcagagtgtttcgctcagcactaccccagtgtagatcaggtcgatgagtcaccgcattccccacgggcgaccgtggcggtggctgcgttggcggcctgcccatggggaaacccatgggacgctctaatacagacatggtgcgaagagtctattgagctagttggtagtcctccggcccctgaatgcggctaatcctaactgcggagcacacaccctcaagccagagggcagtgtgtcgtaacgggcaactctgcagcggaaccgactactttgggtgtccgtgtttcattttattcctatactggctgcttatggtgacaattgagagatcgttaccatatagctattggattggccatccggtgactaatagagctattatatatccctttgttgggtttataccacttagcttgaaagaggttaaaacattacaattcattgttaagttgaatacagcaaaatggtgagcaagggcgaggagctgttcaccggggtggtgcccatcctggtcgagctggacggcgacgtaaacggccacaagttcagcgtgtccggcgagggcgagggcgatgccacctacggcaagctgaccctgaagttcatctgcaccaccggcaagctgcccgtgccctggcccaccctcgtgaccaccctgacctacggcgtgcagtgcttcagccgctaccccgaccacatgaagcagcacgacttcttcaagtccgccatgcccgaaggctacgtccaggagcgcaccatcttcttcaaggacgacggcaactacaagacccgcgccgaggtgaagttcgagggcgacaccctggtgaaccgcatcgagctgaagggcatcgacttcaaggaggacggcaacatcctggggcacaagctggagtacaactacaacagccacaacgtctatatcatggccgacaagcagaagaacggcatcaaggtgaacttcaagatccgccacaacatcgaggacggcagcgtgcagctcgccgaccactaccagcagaacacccccatcggcgacggccccgtgctgctgcccgacaaccactacctgagcacccagtccgccctgagcaaagaccccaacgagaagcgcgatcacatggtcctgctggagttcgtgaccgccgccgggatcactctcggcatggacgagctgtacaagtagttaaaacagcctgtgggttgataaataattgtcccttaaagaagaaattctttaagtggatgctctcaaactcagggaaacctaaatctagttatagacaaggcaatcctgagccaagccgaagtagtaattagtaaggcctagtataccaaaccgcgatatctcttttctag

SEQ ID NO: 58 - RNA, 1639 nt, synthetic construct
  source 1..1639: mol_type = other RNA
gggtcacccgtcgcgcggtttggtatactaggccaacaatagatgacttacaactaatcggaaggtgcagagactcgacgggagctaccctaacgtcaagacgagggtaaagagagagtccaattctcaaagccaataggcagtagcgaaagctgcaagagaatgcccacccacaggcccattgggcgctagcactctggtatcacggtacctttgtgcgcctgttttataccccctcccccaactgtaacttagaagtaacacacaccgatcaacagtcagcgtggcacaccagccacgttttgatcaagcacttctgttaccccggactgagtatcaatagactgctcacgcggttgaaggagaaagcgttcgttatccggccaactacttcgaaaaacctagtaacaccgtggaagttgcagagtgtttcgctcagcactaccccagtgtagatcaggtcgatgagtcaccgcattccccacgggcgaccgtggcggtggctgcgttggcggcctgcccatggggaaacccatgggacgctctaatacagacatggtgcgaagagtctattgagctagttggtagtcctccggcccctgaatgcggctaatcctaactgcggagcacacaccctcaagccagagggcagtgtgtcgtaacgggcaactctgcagcggaaccgactactttgggtgtccgtgtttcattttattcctatactggctgcttatggtgacaattgagagatcgttaccatatagctattggattggccatccggtgactaatagagctattatatatccctttgttgggtttataccacttagcttgaaagaggttaaaacattacaattcattgttaagttgaatacagcaaaatgggggtgcacgaatgtcctgcctggctgtggcttctcctgtccctgctgtcgctccctctgggcctcccagtcctgggcgccccaccacgcctcatctgtgacagccgagtcctggagaggtacctcttggaggccaaggaggccgagaatatcacgacgggctgtgctgaacactgcagcttgaatgagaatatcactgtcccagacaccaaagttaatttctatgcctggaagaggatggaggtcgggcagcaggccgtagaagtctggcagggcctggccctgctgtcggaagctgtcctgcggggccaggccctgttggtcaactcttcccagccgtgggagcccctgcagctgcatgtggataaagccgtcagtggccttcgcagcctcaccactctgcttcgggctctgggagcccagaaggaagccatctcccctccagatgcggcctcagctgctccactccgaacaatcactgctgacactttccgcaaactcttccgagtctactccaatttcctccggggaaagctgaagctgtacacaggggaggcctgcaggacaggggacagatgattaaaacagcctgtgggttgataaataattgtcccttaaagaagaaattctttaagtggatgctctcaaactcagggaaacctaaatctagttatagacaaggcaatcctgagccaagccgaagtagtaattagtaaggcctagtataccaaaccgcgatatctcttttctag

SEQ ID NO: 59 - RNA, 745 nt, synthetic construct
  source 1..745: mol_type = other RNA
gggacatttgcttctgacacaactgtgttcactagcaacctcaaacagacaccatgggagtcaaagttctgtttgccctgatctgcatcgctgtggccgaggccaagcccaccgagaacaacgaagacttcaacatcgtggccgtggccagcaacttcgcgaccacggatctcgatgctgaccgcgggaagttgcccggcaagaagctgccgctggaggtgctcaaagagatggaagccaatgcccggaaagctggctgcaccaggggctgtctgatctgcctgtcccacatcaagtgcacgcccaagatgaagaagttcatcccaggacgctgccacacctacgaaggcgacaaagagtccgcacagggcggcataggcgaggcgatcgtcgacattcctgagattcctgggttcaaggacttggagcccatggagcagttcatcgcacaggtcgatctgtgtgtggactgcacaactggctgcctcaaagggcttgccaacgtgcagtgttctgacctgctcaagaagtggctgccgcaacgctgtgcgacctttgccagcaagatccagggccaggtggacaagatcaagggggccggtggtgactaagctcgctttcttgctgtccaatttctattaaaggttcctttgttccctaagtccaactactaaactgggggatattatgaagggccttgagcatctggattctgcctaataaaaaacatttattttcattgcaa

SEQ ID NO: 60 - RNA, 50 nt, synthetic construct
  source 1..50: mol_type = other RNA
acatttgcttctgacacaactgtgttcactagcaacctcaaacagacacc

SEQ ID NO: 61 - RNA, 134 nt, synthetic construct
  source 1..134: mol_type = other RNA
gctcgctttcttgctgtccaatttctattaaaggttcctttgttccctaagtccaactactaaactgggggatattatgaagggccttgagcatctggattctgcctaataaaaaacatttattttcattgcaa

SEQ ID NO: 62 - RNA, 2394 nt, synthetic construct
  source 1..2394: mol_type = other RNA
ttaaaacagcctgtgggttgatcccacccacaggcccattgggcgctagcactctggtatcacggtacctttgtgcgcctgttttataccccctcccccaactgtaacttagaagtaacacacaccgatcaacagtcagcgtggcacaccagccacgttttgatcaagcacttctgttaccccggactgagtatcaatagactgctcacgcggttgaaggagaaagcgttcgttatccggccaactacttcgaaaaacctagtaacaccgtggaagttgcagagtgtttcgctcagcactaccccagtgtagatcaggtcgatgagtcaccgcattccccacgggcgaccgtggcggtggctgcgttggcggcctgcccatggggaaacccatgggacgctctaatacagacatggtgcgaagagtctattgagctagttggtagtcctccggcccctgaatgcggctaatcctaactgcggagcacacaccctcaagccagagggcagtgtgtcgtaacgggcaactctgcagcggaaccgactactttgggtgtccgtgtttcattttattcctatactggctgcttatggtgacaattgagagatcgttaccatatagctattggattggccatccggtgactaatagagctattatatatccctttgttgggtttataccacttagcttgaaagaggttaaaacattacaattcattgttaagttgaatacagcaaaatggaggacgccaagaacatcaagaagggccccgcccccttctaccccctggaggacggcaccgccggcgagcagctgcacaaggccatgaagcggtacgccctggtgcccggcaccatcgccttcaccgacgcccacatcgaggtggacatcacctacgccgagtacttcgagatgagcgtgcggctggccgaggccatgaagcggtacggcctgaacaccaaccaccggatcgtggtgtgcagcgagaacagcctgcagttcttcatgcccgtgctgggcgccctgttcatcggcgtggccgtggcccccgccaacgacatctacaacgagcgggagctgctgaacagcatgggcatcagccagcccaccgtggtgttcgtgagcaagaagggcctgcagaagatcctgaacgtgcagaagaagctgcccatcatccagaagatcatcatcatggacagcaagaccgactaccagggcttccagagcatgtacaccttcgtgaccagccacctgccccccggcttcaacgagtacgacttcgtgcccgagagcttcgaccgggacaagaccatcgccctgatcatgaacagcagcggcagcaccggcctgcccaagggcgtggccctgccccaccggaccgcctgcgtgcggttcagccacgcccgggaccccatcttcggcaaccagatcatccccgacaccgccatcctgagcgtggtgcccttccaccacggcttcggcatgttcaccaccctgggctacctgatctgcggcttccgggtggtgctgatgtaccggttcgaggaggagctgttcctgcggagcctgcaggactacaagatccagagcgccctgctggtgcccaccctgttcagcttcttcgccaagagcaccctgatcgacaagtacgacctgagcaacctgcacgagatcgccagcggcggcgcccccctgagcaaggaggtgggcgaggccgtggccaagcggttccacctgcccggcatccggcagggctacggcctgaccgagaccaccagcgccatcctgatcacccccgagggcgacgacaagcccggcgccgtgggcaaggtggtgcccttcttcgaggccaaggtggtggacctggacaccggcaagaccctgggcgtgaaccagcggggcgagctgtgcgtgcggggccccatgatcatgagcggctacgtgaacaaccccgaggccaccaacgccctgatcgacaaggacggctggctgcacagcggcgacatcgcctactgggacgaggacgagcacttcttcatcgtggaccggctgaagagcctgatcaagtacaagggctaccaggtggcccccgccgagctggagagcatcctgctgcagcaccccaacatcttcgacgccggcgtggccggcctgcccgacgacgacgccggcgagctgcccgccgccgtggtggtgctggagcacggcaagaccatgaccgagaaggagatcgtggactacgtggccagccaggtgaccaccgccaagaagctgcggggcggcgtggtgttcgtggacgaggtgcccaagggcctgaccggcaagctggacgcccggaagatccgggagatcctgatcaaggccaagaagggcggcaagatcgccgtgtga

SEQ ID NO: 63 - RNA, 2710 nt, synthetic construct
  source 1..2710: mol_type = other RNA
gggtcacccgtcgcgcggtttggtatactaggccaacaatagatgacttacaactaatcggaaggtgcagagactcgacgggagctaccctaacgtcaagacgagggtaaagagagagtccaattctcaaagccaataggcagtagcgaaagctgcaagagaatgcccacccacaggcccattgggcgctagcactctggtatcacggtacctttgtgcgcctgttttataccccctcccccaactgtaacttagaagtaacacacaccgatcaacagtcagcgtggcacaccagccacgttttgatcaagcacttctgttaccccggactgagtatcaatagactgctcacgcggttgaaggagaaagcgttcgttatccggccaactacttcgaaaaacctagtaacaccgtggaagttgcagagtgtttcgctcagcactaccccagtgtagatcaggtcgatgagtcaccgcattccccacgggcgaccgtggcggtggctgcgttggcggcctgcccatggggaaacccatgggacgctctaatacagacatggtgcgaagagtctattgagctagttggtagtcctccggcccctgaatgcggctaatcctaactgcggagcacacaccctcaagccagagggcagtgtgtcgtaacgggcaactctgcagcggaaccgactactttgggtgtccgtgtttcattttattcctatactggctgcttatggtgacaattgagagatcgttaccatatagctattggattggccatccggtgactaatagagctattatatatccctttgttgggtttataccacttagcttgaaagaggttaaaacattacaattcattgttaagttgaatacagcaaaatggaggacgccaagaacatcaagaagggccccgcccccttctaccccctggaggacggcaccgccggcgagcagctgcacaaggccatgaagcggtacgccctggtgcccggcaccatcgccttcaccgacgcccacatcgaggtggacatcacctacgccgagtacttcgagatgagcgtgcggctggccgaggccatgaagcggtacggcctgaacaccaaccaccggatcgtggtgtgcagcgagaacagcctgcagttcttcatgcccgtgctgggcgccctgttcatcggcgtggccgtggcccccgccaacgacatctacaacgagcgggagctgctgaacagcatgggcatcagccagcccaccgtggtgttcgtgagcaagaagggcctgcagaagatcctgaacgtgcagaagaagctgcccatcatccagaagatcatcatcatggacagcaagaccgactaccagggcttccagagcatgtacaccttcgtgaccagccacctgccccccggcttcaacgagtacgacttcgtgcccgagagcttcgaccgggacaagaccatcgccctgatcatgaacagcagcggcagcaccggcctgcccaagggcgtggccctgccccaccggaccgcctgcgtgcggttcagccacgcccgggaccccatcttcggcaaccagatcatccccgacaccgccatcctgagcgtggtgcccttccaccacggcttcggcatgttcaccaccctgggctacctgatctgcggcttccgggtggtgctgatgtaccggttcgaggaggagctgttcctgcggagcctgcaggactacaagatccagagcgccctgctggtgcccaccctgttcagcttcttcgccaagagcaccctgatcgacaagtacgacctgagcaacctgcacgagatcgccagcggcggcgcccccctgagcaaggaggtgggcgaggccgtggccaagcggttccacctgcccggcatccggcagggctacggcctgaccgagaccaccagcgccatcctgatcacccccgagggcgacgacaagcccggcgccgtgggcaaggtggtgcccttcttcgaggccaaggtggtggacctggacaccggcaagaccctgggcgtgaaccagcggggcgagctgtgcgtgcggggccccatgatcatgagcggctacgtgaacaaccccgaggccaccaacgccctgatcgacaaggacggctggctgcacagcggcgacatcgcctactgggacgaggacgagcacttcttcatcgtggaccggctgaagagcctgatcaagtacaagggctaccaggtggcccccgccgagctggagagcatcctgctgcagcaccccaacatcttcgacgccggcgtggccggcctgcccgacgacgacgccggcgagctgcccgccgccgtggtggtgctggagcacggcaagaccatgaccgagaaggagatcgtggactacgtggccagccaggtgaccaccgccaagaagctgcggggcggcgtggtgttcgtggacgaggtgcccaagggcctgaccggcaagctggacgcccggaagatccgggagatcctgatcaaggccaagaagggcggcaagatcgccgtgtgattaaaacagcctgtgggttgataaataattgtcccttaaagaagaaattctttaagtggatgctctcaaactcagggaaacctaaatctagttatagacaaggcaatcctgagccaagccgaagtagtaattagtaaggcctagtataccaaaccgcgatatctcttttctag

SEQ ID NO: 64 - RNA, 2570 nt, synthetic construct
  source 1..2570: mol_type = other RNA
aaaatccgttgaccttaaacggtcgtgtgggttcaagtccctccacccccacgccggaaacgcaatagccgaaaaacaaaaaacaaaaaaaacaaaaaaaaaaccaaaaaaacaaaacacattaaaacagcctgtgggttgatcccacccacaggcccattgggcgctagcactctggtatcacggtacctttgtgcgcctgttttataccccctcccccaactgtaacttagaagtaacacacaccgatcaacagtcagcgtggcacaccagccacgttttgatcaagcacttctgttaccccggactgagtatcaatagactgctcacgcggttgaaggagaaagcgttcgttatccggccaactacttcgaaaaacctagtaacaccgtggaagttgcagagtgtttcgctcagcactaccccagtgtagatcaggtcgatgagtcaccgcattccccacgggcgaccgtggcggtggctgcgttggcggcctgcccatggggaaacccatgggacgctctaatacagacatggtgcgaagagtctattgagctagttggtagtcctccggcccctgaatgcggctaatcctaactgcggagcacacaccctcaagccagagggcagtgtgtcgtaacgggcaactctgcagcggaaccgactactttgggtgtccgtgtttcattttattcctatactggctgcttatggtgacaattgagagatcgttaccatatagctattggattggccatccggtgactaatagagctattatatatccctttgttgggtttataccacttagcttgaaagaggttaaaacattacaattcattgttaagttgaatacagcaaaatggaggacgccaagaacatcaagaagggccccgcccccttctaccccctggaggacggcaccgccggcgagcagctgcacaaggccatgaagcggtacgccctggtgcccggcaccatcgccttcaccgacgcccacatcgaggtggacatcacctacgccgagtacttcgagatgagcgtgcggctggccgaggccatgaagcggtacggcctgaacaccaaccaccggatcgtggtgtgcagcgagaacagcctgcagttcttcatgcccgtgctgggcgccctgttcatcggcgtggccgtggcccccgccaacgacatctacaacgagcgggagctgctgaacagcatgggcatcagccagcccaccgtggtgttcgtgagcaagaagggcctgcagaagatcctgaacgtgcagaagaagctgcccatcatccagaagatcatcatcatggacagcaagaccgactaccagggcttccagagcatgtacaccttcgtgaccagccacctgccccccggcttcaacgagtacgacttcgtgcccgagagcttcgaccgggacaagaccatcgccctgatcatgaacagcagcggcagcaccggcctgcccaagggcgtggccctgccccaccggaccgcctgcgtgcggttcagccacgcccgggaccccatcttcggcaaccagatcatccccgacaccgccatcctgagcgtggtgcccttccaccacggcttcggcatgttcaccaccctgggctacctgatctgcggcttccgggtggtgctgatgtaccggttcgaggaggagctgttcctgcggagcctgcaggactacaagatccagagcgccctgctggtgcccaccctgttcagcttcttcgccaagagcaccctgatcgacaagtacgacctgagcaacctgcacgagatcgccagcggcggcgcccccctgagcaaggaggtgggcgaggccgtggccaagcggttccacctgcccggcatccggcagggctacggcctgaccgagaccaccagcgccatcctgatcacccccgagggcgacgacaagcccggcgccgtgggcaaggtggtgcccttcttcgaggccaaggtggtggacctggacaccggcaagaccctgggcgtgaaccagcggggcgagctgtgcgtgcggggccccatgatcatgagcggctacgtgaacaaccccgaggccaccaacgccctgatcgacaaggacggctggctgcacagcggcgacatcgcctactgggacgaggacgagcacttcttcatcgtggaccggctgaagagcctgatcaagtacaagggctaccaggtggcccccgccgagctggagagcatcctgctgcagcaccccaacatcttcgacgccggcgtggccggcctgcccgacgacgacgccggcgagctgcccgccgccgtggtggtgctggagcacggcaagaccatgaccgagaaggagatcgtggactacgtggccagccaggtgaccaccgccaagaagctgcggggcggcgtggtgttcgtggacgaggtgcccaagggcctgaccggcaagctggacgcccggaagatccgggagatcctgatcaaggccaagaagggcggcaagatcgccgtgtgaaaaaaacaaaaaacaaaacggctattatgcgttaccggcgagacgctacggactt

SEQ ID NO: 65 - RNA, 2885 nt, synthetic construct
  source 1..2885: mol_type = other RNA
gggagaccctcgaccgtcgattgtccactggtcaacaatagatgacttacaactaatcggaaggtgcagagactcgacgggagctaccctaacgtcaagacgagggtaaagagagagtccaattctcaaagccaataggcagtagcgaaagctgcaagagaatgaaaatccgttgaccttaaacggtcgtgtgggttcaagtccctccacccccacgccggaaacgcaatagccgaaaaacaaaaaacaaaaaaaacaaaaaaaaaaccaaaaaaacaaaacacattaaaacagcctgtgggttgatcccacccacaggcccattgggcgctagcactctggtatcacggtacctttgtgcgcctgttttataccccctcccccaactgtaacttagaagtaacacacaccgatcaacagtcagcgtggcacaccagccacgttttgatcaagcacttctgttaccccggactgagtatcaatagactgctcacgcggttgaaggagaaagcgttcgttatccggccaactacttcgaaaaacctagtaacaccgtggaagttgcagagtgtttcgctcagcactaccccagtgtagatcaggtcgatgagtcaccgcattccccacgggcgaccgtggcggtggctgcgttggcggcctgcccatggggaaacccatgggacgctctaatacagacatggtgcgaagagtctattgagctagttggtagtcctccggcccctgaatgcggctaatcctaactgcggagcacacaccctcaagccagagggcagtgtgtcgtaacgggcaactctgcagcggaaccgactactttgggtgtccgtgtttcattttattcctatactggctgcttatggtgacaattgagagatcgttaccatatagctattggattggccatccggtgactaatagagctattatatatccctttgttgggtttataccacttagcttgaaagaggttaaaacattacaattcattgttaagttgaatacagcaaaatggaggacgccaagaacatcaagaagggccccgcccccttctaccccctggaggacggcaccgccggcgagcagctgcacaaggccatgaagcggtacgccctggtgcccggcaccatcgccttcaccgacgcccacatcgaggtggacatcacctacgccgagtacttcgagatgagcgtgcggctggccgaggccatgaagcggtacggcctgaacaccaaccaccggatcgtggtgtgcagcgagaacagcctgcagttcttcatgcccgtgctgggcgccctgttcatcggcgtggccgtggcccccgccaacgacatctacaacgagcgggagctgctgaacagcatgggcatcagccagcccaccgtggtgttcgtgagcaagaagggcctgcagaagatcctgaacgtgcagaagaagctgcccatcatccagaagatcatcatcatggacagcaagaccgactaccagggcttccagagcatgtacaccttcgtgaccagccacctgccccccggcttcaacgagtacgacttcgtgcccgagagcttcgaccgggacaagaccatcgccctgatcatgaacagcagcggcagcaccggcctgcccaagggcgtggccctgccccaccggaccgcctgcgtgcggttcagccacgcccgggaccccatcttcggcaaccagatcatccccgacaccgccatcctgagcgtggtgcccttccaccacggcttcggcatgttcaccaccctgggctacctgatctgcggcttccgggtggtgctgatgtaccggttcgaggaggagctgttcctgcggagcctgcaggactacaagatccagagcgccctgctggtgcccaccctgttcagcttcttcgccaagagcaccctgatcgacaagtacgacctgagcaacctgcacgagatcgccagcggcggcgcccccctgagcaaggaggtgggcgaggccgtggccaagcggttccacctgcccggcatccggcagggctacggcctgaccgagaccaccagcgccatcctgatcacccccgagggcgacgacaagcccggcgccgtgggcaaggtggtgcccttcttcgaggccaaggtggtggacctggacaccggcaagaccctgggcgtgaaccagcggggcgagctgtgcgtgcggggccccatgatcatgagcggctacgtgaacaaccccgaggccaccaacgccctgatcgacaaggacggctggctgcacagcggcgacatcgcctactgggacgaggacgagcacttcttcatcgtggaccggctgaagagcctgatcaagtacaagggctaccaggtggcccccgccgagctggagagcatcctgctgcagcaccccaacatcttcgacgccggcgtggccggcctgcccgacgacgacgccggcgagctgcccgccgccgtggtggtgctggagcacggcaagaccatgaccgagaaggagatcgtggactacgtggccagccaggtgaccaccgccaagaagctgcggggcggcgtggtgttcgtggacgaggtgcccaagggcctgaccggcaagctggacgcccggaagatccgggagatcctgatcaaggccaagaagggcggcaagatcgccgtgtgaaaaaaacaaaaaacaaaacggctattatgcgttaccggcgagacgctacggacttaaataattgagccttaaagaagaaattctttaagtggatgctctcaaactcagggaaacctaaatctagttatagacaaggcaatcctgagccaagccgaagtagtaattagtaagaccagtggacaatcgacggataacagcatatctag

SEQ ID NO: 66 - RNA, 1323 nt, synthetic construct
  source 1..1323: mol_type = other RNA
ttaaaacagcctgtgggttgatcccacccacaggcccattgggcgctagcactctggtatcacggtacctttgtgcgcctgttttataccccctcccccaactgtaacttagaagtaacacacaccgatcaacagtcagcgtggcacaccagccacgttttgatcaagcacttctgttaccccggactgagtatcaatagactgctcacgcggttgaaggagaaagcgttcgttatccggccaactacttcgaaaaacctagtaacaccgtggaagttgcagagtgtttcgctcagcactaccccagtgtagatcaggtcgatgagtcaccgcattccccacgggcgaccgtggcggtggctgcgttggcggcctgcccatggggaaacccatgggacgctctaatacagacatggtgcgaagagtctattgagctagttggtagtcctccggcccctgaatgcggctaatcctaactgcggagcacacaccctcaagccagagggcagtgtgtcgtaacgggcaactctgcagcggaaccgactactttgggtgtccgtgtttcattttattcctatactggctgcttatggtgacaattgagagatcgttaccatatagctattggattggccatccggtgactaatagagctattatatatccctttgttgggtttataccacttagcttgaaagaggttaaaacattacaattcattgttaagttgaatacagcaaaatgggggtgcacgaatgtcctgcctggctgtggcttctcctgtccctgctgtcgctccctctgggcctcccagtcctgggcgccccaccacgcctcatctgtgacagccgagtcctggagaggtacctcttggaggccaaggaggccgagaatatcacgacgggctgtgctgaacactgcagcttgaatgagaatatcactgtcccagacaccaaagttaatttctatgcctggaagaggatggaggtcgggcagcaggccgtagaagtctggcagggcctggccctgctgtcggaagctgtcctgcggggccaggccctgttggtcaactcttcccagccgtgggagcccctgcagctgcatgtggataaagccgtcagtggccttcgcagcctcaccactctgcttcgggctctgggagcccagaaggaagccatctcccctccagatgcggcctcagctgctccactccgaacaatcactgctgacactttccgcaaactcttccgagtctactccaatttcctccggggaaagctgaagctgtacacaggggaggcctgcaggacaggggacagatga

SEQ ID NO: 67 - RNA, 1814 nt, synthetic construct
  source 1..1814: mol_type = other RNA
gggagaccctcgaccgtcgattgtccactggtcaacaatagatgacttacaactaatcggaaggtgcagagactcgacgggagctaccctaacgtcaagacgagggtaaagagagagtccaattctcaaagccaataggcagtagcgaaagctgcaagagaatgaaaatccgttgaccttaaacggtcgtgtgggttcaagtccctccacccccacgccggaaacgcaatagccgaaaaacaaaaaacaaaaaaaacaaaaaaaaaaccaaaaaaacaaaacacattaaaacagcctgtgggttgatcccacccacaggcccattgggcgctagcactctggtatcacggtacctttgtgcgcctgttttataccccctcccccaactgtaacttagaagtaacacacaccgatcaacagtcagcgtggcacaccagccacgttttgatcaagcacttctgttaccccggactgagtatcaatagactgctcacgcggttgaaggagaaagcgttcgttatccggccaactacttcgaaaaacctagtaacaccgtggaagttgcagagtgtttcgctcagcactaccccagtgtagatcaggtcgatgagtcaccgcattccccacgggcgaccgtggcggtggctgcgttggcggcctgcccatggggaaacccatgggacgctctaatacagacatggtgcgaagagtctattgagctagttggtagtcctccggcccctgaatgcggctaatcctaactgcggagcacacaccctcaagccagagggcagtgtgtcgtaacgggcaactctgcagcggaaccgactactttgggtgtccgtgtttcattttattcctatactggctgcttatggtgacaattgagagatcgttaccatatagctattggattggccatccggtgactaatagagctattatatatccctttgttgggtttataccacttagcttgaaagaggttaaaacattacaattcattgttaagttgaatacagcaaaatgggggtgcacgaatgtcctgcctggctgtggcttctcctgtccctgctgtcgctccctctgggcctcccagtcctgggcgccccaccacgcctcatctgtgacagccgagtcctggagaggtacctcttggaggccaaggaggccgagaatatcacgacgggctgtgctgaacactgcagcttgaatgagaatatcactgtcccagacaccaaagttaatttctatgcctggaagaggatggaggtcgggcagcaggccgtagaagtctggcagggcctggccctgctgtcggaagctgtcctgcggggccaggccctgttggtcaactcttcccagccgtgggagcccctgcagctgcatgtggataaagccgtcagtggccttcgcagcctcaccactctgcttcgggctctgggagcccagaaggaagccatctcccctccagatgcggcctcagctgctccactccgaacaatcactgctgacactttccgcaaactcttccgagtctactccaatttcctccggggaaagctgaagctgtacacaggggaggcctgcaggacaggggacagatgaaaaaaacaaaaaacaaaacggctattatgcgttaccggcgagacgctacggacttaaataattgagccttaaagaagaaattctttaagtggatgctctcaaactcagggaaacctaaatctagttatagacaaggcaatcctgagccaagccgaagtagtaattagtaagaccagtggacaatcgacggataacagcatatctag

SEQ ID NO: 68 - RNA, 741 nt, synthetic construct; identical to SEQ ID NO: 1
  source 1..741: mol_type = other RNA

SEQ ID NO: 69 - RNA, 50 nt, synthetic construct
  source 1..50: mol_type = other RNA
cggactgagtatcaatagactgctcacgcggttgaaggagaaagcgttcg

SEQ ID NO: 70 - RNA, 558 nt, synthetic construct; identical to SEQ ID NO: 3
  source 1..558: mol_type = other RNA

SEQ ID NO: 71 - RNA, 1299 nt, synthetic construct; identical to SEQ ID NO: 4
  source 1..1299: mol_type = other RNA

SEQ ID NO: 72 - RNA, 1299 nt, synthetic construct
  source 1..1299: mol_type = other RNA
cacgcggttgaaggagaaagcgttcgttatccggccaactacttcgaaaaacctagtaacaccgtggaagttgcagagtgtttcgctcagcactaccccagtgtagatcaggtcgatgagtcaccgcattccccacgggcgaccgtggcggtggctgcgttggcggcctgcccatggggaaacccatgggacgctctaatacagacatggtgcgaagagtctattgagctagttggtagtcctccggcccctgaatgcggctaatcctaactgcggagcacacaccctcaagccagagggcagtgtgtcgtaacgggcaactctgcagcggaaccgactactttgggtgtccgtgtttcattttattcctatactggctgcttatggtgacaattgagagatcgttaccatatagctattggattggccatccggtgactaatagagctattatatatccctttgttgggtttataccacttagcttgaaagaggttaaaacattacaattcattgttaagttgaatacagcaaaatgggagtcaaagttctgtttgccctgatctgcatcgctgtggccgaggccaagcccaccgagaacaacgaagacttcaacatcgtggccgtggccagcaacttcgcgaccacggatctcgatgctgaccgcgggaagttgcccggcaagaagctgccgctggaggtgctcaaagagatggaagccaatgcccggaaagctggctgcaccaggggctgtctgatctgcctgtcccacatcaagtgcacgcccaagatgaagaagttcatcccaggacgctgccacacctacgaaggcgacaaagagtccgcacagggcggcataggcgaggcgatcgtcgacattcctgagattcctgggttcaaggacttggagcccatggagcagttcatcgcacaggtcgatctgtgtgtggactgcacaactggctgcctcaaagggcttgccaacgtgcagtgttctgacctgctcaagaagtggctgccgcaacgctgtgcgacctttgccagcaagatccagggccaggtggacaagatcaagggggccggtggtgactaattaaaacagcctgtgggttgatcccacccacaggcccattgggcgctagcactctggtatcacggtacctttgtgcgcctgttttataccccctcccccaactgtaacttagaagtaacacacaccgatcaacagtcagcgtggcacaccagccacgttttgatcaagcacttctgttaccccggactgagtatcaatagactgct

SEQ ID NO: 73 - RNA, 165 nt, synthetic construct; identical to SEQ ID NO: 6
  source 1..165: mol_type = other RNA

SEQ ID NO: 74 - RNA, 151 nt, synthetic construct
  source 1..151: mol_type = other RNA
aaataattggcccttaaagaagaaattctttaagtggatgctctcaaactcagggaaacctaaatctagttatagacaaggcaatcctgagccaagccgaagtagtaattagtaaggcctagtataccaaaccgcgatatctcttttctag

SEQ ID NO: 75 - RNA, 1615 nt, synthetic construct
  source 1..1615: mol_type = other RNA
gggtcacccgtcgcgcggtttggtatactaggccaacaatagatgacttacaactaatcggaaggtgcagagactcgacgggagctaccctaacgtcaagacgagggtaaagagagagtccaattctcaaagccaataggcagtagcgaaagctgcaagagaatgcacgcggttgaaggagaaagcgttcgttatccggccaactacttcgaaaaacctagtaacaccgtggaagttgcagagtgtttcgctcagcactaccccagtgtagatcaggtcgatgagtcaccgcattccccacgggcgaccgtggcggtggctgcgttggcggcctgcccatggggaaacccatgggacgctctaatacagacatggtgcgaagagtctattgagctagttggtagtcctccggcccctgaatgcggctaatcctaactgcggagcacacaccctcaagccagagggcagtgtgtcgtaacgggcaactctgcagcggaaccgactactttgggtgtccgtgtttcattttattcctatactggctgcttatggtgacaattgagagatcgttaccatatagctattggattggccatccggtgactaatagagctattatatatccctttgttgggtttataccacttagcttgaaagaggttaaaacattacaattcattgttaagttgaatacagcaaaatgggagtcaaagttctgtttgccctgatctgcatcgctgtggccgaggccaagcccaccgagaacaacgaagacttcaacatcgtggccgtggccagcaacttcgcgaccacggatctcgatgctgaccgcgggaagttgcccggcaagaagctgccgctggaggtgctcaaagagatggaagccaatgcccggaaagctggctgcaccaggggctgtctgatctgcctgtcccacatcaagtgcacgcccaagatgaagaagttcatcccaggacgctgccacacctacgaaggcgacaaagagtccgcacagggcggcataggcgaggcgatcgtcgacattcctgagattcctgggttcaaggacttggagcccatggagcagttcatcgcacaggtcgatctgtgtgtggactgcacaactggctgcctcaaagggcttgccaacgtgcagtgttctgacctgctcaagaagtggctgccgcaacgctgtgcgacctttgccagcaagatccagggccaggtggacaagatcaagggggccggtggtgactaattaaaacagcctgtgggttgatcccacccacaggcccattgggcgctagcactctggtatcacggtacctttgtgcgcctgttttataccccctcccccaactgtaacttagaagtaacacacaccgatcaacagtcagcgtggcacaccagccacgttttgatcaagcacttctgttaccccggactgagtatcaatagactgctaaataattggcccttaaagaagaaattctttaagtggatgctctcaaactcagggaaacctaaatctagttatagacaaggcaatcctgagccaagccgaagtagtaattagtaaggcctagtataccaaaccgcgatatctcttttctag

SEQ ID NO: 76 - RNA, 151 nt, synthetic construct; identical to SEQ ID NO: 9
  source 1..151: mol_type = other RNA

SEQ ID NO: 77 - RNA, 37 nt, synthetic construct
  source 1..37: mol_type = other RNA
gcagttcatcgcacaggtcgatctgtgtgtggactgc

SEQ ID NO: 78 - RNA, 558 nt, synthetic construct
  source 1..558: mol_type = other RNA
atgggcgtcaaggtgctctttgccctgatctgcatcgcggtggcggaggcgaagcccacggagaacaatgaggacttcaacattgttgccgtggcttcgaacttcgccaccactgacttagatgcagatcggggcaagcttccggggaagaagcttcccctggaagttctcaaggagatggaggcgaacgctcgcaaggccggttgcacccgtgggtgcttgatttgtctctctcatatcaagtgcacccccaagatgaagaaattcatccctgggcggtgtcacacttatgagggagacaaagagagcgcccagggtgggatcggcgaggcgatcgtcgacatccctgagatccctgggttcaaggaccttgagcccatggagcagttcatcgcacaggtggacctgtgcgtggactgcaccactggatgtttgaagggactggccaacgttcagtgcagcgacttgctgaagaagtggctgcctcagcgttgtgccacgttcgcttcaaagatccagggtcaggtcgacaagatcaagggcgccggcggcgattaa

SEQ ID NO: 79 - RNA, 37 nt, synthetic construct
  source 1..37: mol_type = other RNA
gcagttcatcgcacaggtggacctgtgcgtggactgc

SEQ ID NO: 80 - RNA, 1615 nt, synthetic construct
  source 1..1615: mol_type = other RNA
gggtcacccgtcgcgcggtttggtatactaggccaacaatagatgacttacaactaatcggaaggtgcagagactcgacgggagctaccctaacgtcaagacgagggtaaagagagagtccaattctcaaagccaataggcagtagcgaaagctgcaagagaatgcgatctgtgtgtggactgcacaactggctgcctcaaagggcttgccaacgtgcagtgttctgacctgctcaagaagtggctgccgcaacgctgtgcgacctttgccagcaagatccagggccaggtggacaagatcaagggggccggtggtgactaattaaaacagcctgtgggttgatcccacccacaggcccattgggcgctagcactctggtatcacggtacctttgtgcgcctgttttataccccctcccccaactgtaacttagaagtaacacacaccgatcaacagtcagcgtggcacaccagccacgttttgatcaagcacttctgttaccccggactgagtatcaatagactgctcacgcggttgaaggagaaagcgttcgttatccggccaactacttcgaaaaacctagtaacaccgtggaagttgcagagtgtttcgctcagcactaccccagtgtagatcaggtcgatgagtcaccgcattccccacgggcgaccgtggcggtggctgcgttggcggcctgcccatggggaaacccatgggacgctctaatacagacatggtgcgaagagtctattgagctagttggtagtcctccggcccctgaatgcggctaatcctaactgcggagcacacaccctcaagccagagggcagtgtgtcgtaacgggcaactctgcagcggaaccgactactttgggtgtccgtgtttcattttattcctatactggctgcttatggtgacaattgagagatcgttaccatatagctattggattggccatccggtgactaatagagctattatatatccctttgttgggtttataccacttagcttgaaagaggttaaaacattacaattcattgttaagttgaatacagcaaaatgggagtcaaagttctgtttgccctgatctgcatcgctgtggccgaggccaagcccaccgagaacaacgaagacttcaacatcgtggccgtggccagcaacttcgcgaccacggatctcgatgctgaccgcgggaagttgcccggcaagaagctgccgctggaggtgctcaaagagatggaagccaatgcccggaaagctggctgcaccaggggctgtctgatctgcctgtcccacatcaagtgcacgcccaagatgaagaagttcatcccaggacgctgccacacctacgaaggcgacaaagagtccgcacagggcggcataggcgaggcgatcgtcgacattcctgagattcctgggttcaaggacttggagcccatggagcagttcatcgcacaggtaaataattgccccttaaagaagaaattctttaagtggatgctctcaaactcagggaaacctaaatctagttatagacaaggcaatcctgagccaagccgaagtagtaattagtaaggcctagtataccaaaccgcgatatctcttttctag

SEQ ID NO: 81 - RNA, 1615 nt, synthetic construct
  source 1..1615: mol_type = other RNA
gggtcacccgtcgcgcggtttggtatactaggccaacaatagatgacttacaactaatcggaaggtgcagagactcgacgggagctaccctaacgtcaagacgagggtaaagagagagtccaattctcaaagccaataggcagtagcgaaagctgcaagagaatgggacctgtgcgtggactgcaccactggatgtttgaagggactggccaacgttcagtgcagcgacttgctgaagaagtggctgcctcagcgttgtgccacgttcgcttcaaagatccagggtcaggtcgacaagatcaagggcgccggcggcgattaattaaaacagcctgtgggttgatcccacccacaggcccattgggcgctagcactctggtatcacggtacctttgtgcgcctgttttataccccctcccccaactgtaacttagaagtaacacacaccgatcaacagtcagcgtggcacaccagccacgttttgatcaagcacttctgttaccccggactgagtatcaatagactgctcacgcggttgaaggagaaagcgttcgttatccggccaactacttcgaaaaacctagtaacaccgtggaagttgcagagtgtttcgctcagcactaccccagtgtagatcaggtcgatgagtcaccgcattccccacgggcgaccgtggcggtggctgcgttggcggcctgcccatggggaaacccatgggacgctctaatacagacatggtgcgaagagtctattgagctagttggtagtcctccggcccctgaatgcggctaatcctaactgcggagcacacaccctcaagccagagggcagtgtgtcgtaacgggcaactctgcagcggaaccgactactttgggtgtccgtgtttcattttattcctatactggctgcttatggtgacaattgagagatcgttaccatatagctattggattggccatccggtgactaatagagctattatatatccctttgttgggtttataccacttagcttgaaagaggttaaaacattacaattcattgttaagttgaatacagcaaaatgggcgtcaaggtgctctttgccctgatctgcatcgcggtggcggaggcgaagcccacggagaacaatgaggacttcaacattgttgccgtggcttcgaacttcgccaccactgacttagatgcagatcggggcaagcttccggggaagaagcttcccctggaagttctcaaggagatggaggcgaacgctcgcaaggccggttgcacccgtgggtgcttgatttgtctctctcatatcaagtgcacccccaagatgaagaaattcatccctgggcggtgtcacacttatgagggagacaaagagagcgcccagggtgggatcggcgaggcgatcgtcgacatccctgagatccctgggttcaaggaccttgagcccatggagcagttcatcgcacaggtaaataattgccccttaaagaagaaattctttaagtggatgctctcaaactcagggaaacctaaatctagttatagacaaggcaatcctgagccaagccgaagtagtaattagtaaggcctagtataccaaaccgcgatatctcttttctag

SEQ ID NO: 82 - RNA, 1615 nt, synthetic construct
  source 1..1615: mol_type = other RNA
gggtcacccgtcgcgcggtttggtatactaggccaacaatagatgacttacaactaatcggaaggtgcagagactcgacgggagctaccctaacgtcaagacgagggtaaagagagagtccaattctcaaagccaataggcagtagcgaaagctgcaagagaatgagactgctcacgcggttgaaggagaaagcgttcgttatccggccaactacttcgaaaaacctagtaacaccgtggaagttgcagagtgtttcgctcagcactaccccagtgtagatcaggtcgatgagtcaccgcattccccacgggcgaccgtggcggtggctgcgttggcggcctgcccatggggaaacccatgggacgctctaatacagacatggtgcgaagagtctattgagctagttggtagtcctccggcccctgaatgcggctaatcctaactgcggagcacacaccctcaagccagagggcagtgtgtcgtaacgggcaactctgcagcggaaccgactactttgggtgtccgtgtttcattttattcctatactggctgcttatggtgacaattgagagatcgttaccatatagctattggattggccatccggtgactaatagagctattatatatccctttgttgggtttataccacttagcttgaaagaggttaaaacattacaattcattgttaagttgaatacagcaaaatgggagtcaaagttctgtttgccctgatctgcatcgctgtggccgaggccaagcccaccgagaacaacgaagacttcaacatcgtggccgtggccagcaacttcgcgaccacggatctcgatgctgaccgcgggaagttgcccggcaagaagctgccgctggaggtgctcaaagagatggaagccaatgcccggaaagctggctgcaccaggggctgtctgatctgcctgtcccacatcaagtgcacgcccaagatgaagaagttcatcccaggacgctgccacacctacgaaggcgacaaagagtccgcacagggcggcataggcgaggcgatcgtcgacattcctgagattcctgggttcaaggacttggagcccatggagcagttcatcgcacaggtcgatctgtgtgtggactgcacaactggctgcctcaaagggcttgccaacgtgcagtgttctgacctgctcaagaagtggctgccgcaacgctgtgcgacctttgccagcaagatccagggccaggtggacaagatcaagggggccggtggtgactaattaaaacagcctgtgggttgatcccacccacaggcccattgggcgctagcactctggtatcacggtacctttgtgcgcctgttttataccccctcccccaactgtaacttagaagtaacacacaccgatcaacagtcagcgtggcacaccagccacgttttgatcaagcacttctgttaccccggactgagtatcaataaataattgttccttaaagaagaaattctttaagtggatgctctcaaactcagggaaacctaaatctagttatagacaaggcaatcctgagccaagccgaagtagtaattagtaaggcctagtataccaaaccgcgatatctcttttctag

SEQ ID NO: 83 - DNA, 20 bp, synthetic construct
  source 1..20: mol_type = other DNA
ggcattggcttccatctctt

SEQ ID NO: 84 - DNA, 21 bp, synthetic construct
  source 1..21: mol_type = other DNA
cctccatctccttgagaactt

SEQ ID NO: 85 - DNA, 22 bp, synthetic construct
  source 1..22: mol_type = other DNA
aagaagttcatcccaggacgct

SEQ ID NO: 86 - DNA, 20 bp, synthetic construct
  source 1..20: mol_type = other DNA
ggccacgatgttgaagtctt

SEQ ID NO: 87 - DNA, 24 bp, synthetic construct
  source 1..24: mol_type = other DNA
atatagctattggattggccatcc

SEQ ID NO: 88 - DNA, 19 bp, synthetic construct
  source 1..19: mol_type = other DNA
cttcaaccgcgtgagcagt

SEQ ID NO: 89 - RNA, 1618 nt, synthetic construct
  source 1..1618: mol_type = other RNA
gggtcacccgtcgcgcggtttggtatactaggccaacaatagatgacttacaactaatcggaaggtgcagagactcgacgggagctaccctaacgtcaagacgagggtaaagagagagtccaattctcaaagccaataggcagtagcgaaagctgcaagagaatggattgttatcataaagcgaattggattggccatccggtgaaagcgagacttactatttacttacttgttggacttaccacacttaatacatttattctaggtgtcacttgtatagcaattagaatcaaacagttgcatcataatgggagtcaaagttctgtttgccctgatctgcatcgctgtggccgaggccaagcccaccgagaacaacgaagacttcaacatcgtggccgtggccagcaacttcgcgaccacggatctcgatgctgaccgcgggaagttgcccggcaagaagctgccgctggaggtgctcaaagagatggaagccaatgcccggaaagctggctgcaccaggggctgtctgatctgcctgtcccacatcaagtgcacgcccaagatgaagaagttcatcccaggacgctgccacacctacgaaggcgacaaagagtccgcacagggcggcataggcgaggcgatcgtcgacattcctgagattcctgggttcaaggacttggagcccatggagcagttcatcgcacaggtcgatctgtgtgtggactgcacaactggctgcctcaaagggcttgccaacgtgcagtgttctgacctgctcaagaagtggctgccgcaacgctgtgcgacctttgccagcaagatccagggccaggtggacaagatcaagggggccggtggtgactaattaaaacagctctggggttgtacccaccccagaggcccacgtggcggctagtactccggtattacggtacccttgtacgcctgttttatactccctccctcgtaacttagaagcacaaaaccaagttcaatagaagggggtgcaaaccagtaccaccacgaacaagcatttctgtttccccggtgatgttgtatagactgcccgcgcggttgaaagcaacggatccgttacccgctcaagtacttcgagaagcctagtattaccttggaatcttcgatgcgttgcgttcagcactcgaccctggagtgtagcttaggctgatgagtctggacgtccctcaccggtgacggtggtccaggctgcgttggcggcctacctatggctaacgccataggacgctagttgtgaacaaggtgtgaagagcctattgagctacttgagagtcctccggcccctgaatgcggctaatcctaaccatggagcaggcggtcacagaccagtgactagcttgtcgtaatgcgcaagtctatggcggaaccgactactttgggtgtccgtgtttccttttatttttattatggctgcttatggtgacaatcattaaataattgatccttaaagaagaaattctttaagtggatgctctcaaactcagggaaacctaaatctagttatagacaaggcaatcctgagccaagccgaagtagtaattagtaaggcctagtataccaaaccgcgatatctcttttctag

SEQ ID NO: 90 - RNA, 1639 nt, synthetic construct
  source 1..1639: mol_type = other RNA
gggtcacccgtcgcgcggtttggtatactaggccaacaatagatgacttacaactaatcggaaggtgcagagactcgacgggagctaccctaacgtcaagacgagggtaaagagagagtccaattctcaaagccaataggcagtagcgaaagctgcaagagaatggtcctgcggggccaggccctgttggtcaactcttcccagccgtgggagcccctgcagctgcatgtggataaagccgtcagtggccttcgcagcctcaccactctgcttcgggctctgggagcccagaaggaagccatctcccctccagatgcggcctcagctgctccactccgaacaatcactgctgacactttccgcaaactcttccgagtctactccaatttcctccggggaaagctgaagctgtacacaggggaggcctgcaggacaggggacagatgattaaaacagcctgtgggttgatcccacccacaggcccattgggcgctagcactctggtatcacggtacctttgtgcgcctgttttataccccctcccccaactgtaacttagaagtaacacacaccgatcaacagtcagcgtggcacaccagccacgttttgatcaagcacttctgttaccccggactgagtatcaatagactgctcacgcggttgaaggagaaagcgttcgttatccggccaactacttcgaaaaacctagtaacaccgtggaagttgcagagtgtttcgctcagcactaccccagtgtagatcaggtcgatgagtcaccgcattccccacgggcgaccgtggcggtggctgcgttggcggcctgcccatggggaaacccatgggacgctctaatacagacatggtgcgaagagtctattgagctagttggtagtcctccggcccctgaatgcggctaatcctaactgcggagcacacaccctcaagccagagggcagtgtgtcgtaacgggcaactctgcagcggaaccgactactttgggtgtccgtgtttcattttattcctatactggctgcttatggtgacaattgagagatcgttaccatatagctattggattggccatccggtgactaatagagctattatatatccctttgttgggtttataccacttagcttgaaagaggttaaaacattacaattcattgttaagttgaatacagcaaaatgggggtgcacgaatgtcctgcctggctgtggcttctcctgtccctgctgtcgctccctctgggcctcccagtcctgggcgccccaccacgcctcatctgtgacagccgagtcctggagaggtacctcttggaggccaaggaggccgagaatatcacgacgggctgtgctgaacactgcagcttgaatgagaatatcactgtcccagacaccaaagttaatttctatgcctggaagaggatggaggtcgggcagcaggccgtagaagtctggcagggcctggccctgctgtcggaagctaaataattggcccttaaagaagaaattctttaagtggatgctctcaaactcagggaaacctaaatctagttatagacaaggcaatcctgagccaagccgaagtagtaattagtaaggcctagtataccaaaccgcgatatctcttttctag